European Patent Specification EP 3 224 274 B1, published February 14, 2024. Title: MUTANT PORES. Applicant: VIB VZW VRIJE UNIVERSITEIT BRUSSEL STEFAN HOWORKA OXFORD NANOPORE TECHNOLOGIES LIMITED. The sequence listing filed with the application follows.

SEQUENCE LISTING (450 sequences)

SEQ ID NO: 1 - protein, 277 aa, Escherichia coli
MQRLFLLVAVMLLSGCLTAPPKEAARPTLMPRAQSYKDLTHLPAPTGKIFVSVYNIQDETGQFKPYPASNFSTAVPQSATAMLVTALKDSRWFIPLERQGLQNLLNERKIIRAAQENGTVAINNRIPLQSLTAANIMVEGSIIGYESNVKSGGVGARYFGIGADTQYQLDQIAVNLRVVNVSTGEILSSVNTSKTILSYEVQAGVFRFIDYQRLLEGEVGYTSNEPVMLCLMSAIETGVIFLINDGIDRGLWDLQNKAERQNDILVKYRHMSVPPES

SEQ ID NO: 2 - DNA, 834 bp, Escherichia coli
atgcagcgcttatttcttttggttgccgtcatgttactgagcggatgcttaaccgccccgcctaaagaagccgccagaccgacattaatgcctcgtgctcagagctacaaagatttgacccatctgccagcgccgacgggtaaaatctttgtttcggtatacaacattcaggacgaaaccgggcaatttaaaccctacccggcaagtaacttctccactgctgttccgcaaagcgccacggcaatgctggtcacggcactgaaagattctcgctggtttataccgctggagcgccagggcttacaaaacctgcttaacgagcgcaagattattcgtgcggcacaagaaaacggcacggttgccattaataaccgaatcccgctgcaatctttaacggcggcaaatatcatggttgaaggttcgattatcggttatgaaagcaacgtcaaatctggcggggttggggcaagatattttggcatcggtgccgacacgcaataccagctcgatcagattgccgtgaacctgcgcgtcgtcaatgtgagtaccggcgagatcctttcttcggtgaacaccagtaagacgatactttcctatgaagttcaggccggggttttccgctttattgactaccagcgcttgcttgaaggggaagtgggttacacctcgaacgaacctgttatgctgtgcctgatgtcggctatcgaaacaggggtcattttcctgattaatgatggtatcgaccgtggtctgtgggatttgcaaaataaagcagaacggcagaatgacattctggtgaaataccgccatatgtcggttccaccggaatcctga

SEQ ID NO: 3 - protein, 25 aa, Escherichia coli
VYNIQDETGQFKPYPASNFSTAVPQ

SEQ ID NO: 4 - protein, 25 aa, Escherichia coli
VYNIQDETGQFKPYPASNFSTAVPQ

SEQ ID NO: 5 - protein, 25 aa, Escherichia coli
VYNIQDETGQFKPYPASNASTAVPQ

SEQ ID NO: 6 - protein, 25 aa, Escherichia coli
VYNIQDETGQFKPYPASNGSTAVPQ

SEQ ID NO: 7 - protein, 25 aa, Escherichia coli
VYNIQDETGQFKPYPASNVSTAVPQ

SEQ ID NO: 8 - protein, 24 aa, Escherichia coli
VYNIQDETGQFKPYPASNSTAVPQ

SEQ ID NO: 9 - protein, 25 aa, Escherichia coli
VYNIQDETGQFKPYPASAFSTAVPQ

SEQ ID NO: 10 - protein, 25 aa, Escherichia coli
VYNIQDETGQFKPYPASAASTAVPQ

SEQ ID NO: 11 - protein, 25 aa, Escherichia coli
VYNIQDETGQFKPYPASAGSTAVPQ

SEQ ID NO: 12 - protein, 25 aa, Escherichia coli
VYNIQDETGQFKPYPASAVSTAVPQ

SEQ ID NO: 13 - protein, 24 aa, Escherichia coli
VYNIQDETGQFKPYPASASTAVPQ

SEQ ID NO: 14 - protein, 25 aa, Escherichia coli
VYNIQDETGQFKPYPASGFSTAVPQ

SEQ ID NO: 15 - protein, 25 aa, Escherichia coli
VYNIQDETGQFKPYPASGASTAVPQ

SEQ ID NO: 16 - protein, 25 aa, Escherichia coli
VYNIQDETGQFKPYPASGGSTAVPQ

SEQ ID NO: 17 - protein, 25 aa, Escherichia coli
VYNIQDETGQFKPYPASGVSTAVPQ

SEQ ID NO: 18 - protein, 24 aa, Escherichia coli
VYNIQDETGQFKPYPASGSTAVPQ

SEQ ID NO: 19 - protein, 25 aa, Escherichia coli
VYNIQDETGQFKPYPASVFSTAVPQ

SEQ ID NO: 20 - protein, 25 aa, Escherichia coli
VYNIQDETGQFKPYPASVASTAVPQ

SEQ ID NO: 21 - protein, 25 aa, Escherichia coli
VYNIQDETGQFKPYPASVGSTAVPQ

SEQ ID NO: 22 - protein, 25 aa, Escherichia coli
VYNIQDETGQFKPYPASVVSTAVPQ

SEQ ID NO: 23 - protein, 24 aa, Escherichia coli
VYNIQDETGQFKPYPASVSTAVPQ

SEQ ID NO: 24 - protein, 25 aa, Escherichia coli
VYNIQDETGQFKPYPASSFSTAVPQ

SEQ ID NO: 25 - protein, 25 aa, Escherichia coli
VYNIQDETGQFKPYPASSASTAVPQ

SEQ ID NO: 26 - protein, 25 aa, Escherichia coli
VYNIQDETGQFKPYPASSGSTAVPQ

SEQ ID NO: 27 - protein, 25 aa, Escherichia coli
VYNIQDETGQFKPYPASSVSTAVPQ

SEQ ID NO: 28 - protein, 24 aa, Escherichia coli
VYNIQDETGQFKPYPASSSTAVPQ

SEQ ID NO: 29 - protein, 25 aa, Escherichia coli
VYNIQDETGQFKPYPASTFSTAVPQ

SEQ ID NO: 30 - protein, 25 aa, Escherichia coli
VYNIQDETGQFKPYPASTASTAVPQ

SEQ ID NO: 31 - protein, 25 aa, Escherichia coli
VYNIQDETGQFKPYPASTGSTAVPQ

SEQ ID NO: 32 - protein, 25 aa, Escherichia coli
VYNIQDETGQFKPYPASTVSTAVPQ

SEQ ID NO: 33 - protein, 24 aa, Escherichia coli
VYNIQDETGQFKPYPASTSTAVPQ

SEQ ID NO: 34 - protein, 24 aa, Escherichia coli
VYNIQDETGQFKPYPASFSTAVPQ

SEQ ID NO: 35 - protein, 24 aa, Escherichia coli
VYNIQDETGQFKPYPASASTAVPQ

SEQ ID NO: 36 - protein, 24 aa, Escherichia coli
VYNIQDETGQFKPYPASGSTAVPQ

SEQ ID NO: 37 - protein, 24 aa, Escherichia coli
VYNIQDETGQFKPYPASVSTAVPQ

SEQ ID NO: 38 - protein, 23 aa, Escherichia coli
VYNIQDETGQFKPYPASSTAVPQ

SEQ ID NO: 39 - protein, 25 aa, Escherichia coli
VYNIQDETGQFKPAPASNFSTAVPQ

SEQ ID NO: 40 - protein, 25 aa, Escherichia coli
VYNIQDETGQFKPAPASNASTAVPQ

SEQ ID NO: 41 - protein, 25 aa, Escherichia coli
VYNIQDETGQFKPAPASNGSTAVPQ

SEQ ID NO: 42 - protein, 25 aa, Escherichia coli
VYNIQDETGQFKPAPASNVSTAVPQ

SEQ ID NO: 43 - protein, 24 aa, Escherichia coli
VYNIQDETGQFKPAPASNSTAVPQ

SEQ ID NO: 44 - protein, 25 aa, Escherichia coli
VYNIQDETGQFKPAPASAFSTAVPQ

SEQ ID NO: 45 - protein, 25 aa, Escherichia coli
VYNIQDETGQFKPAPASAASTAVPQ

SEQ ID NO: 46 - protein, 25 aa, Escherichia coli
VYNIQDETGQFKPAPASAGSTAVPQ

SEQ ID NO: 47 - protein, 25 aa, Escherichia coli
VYNIQDETGQFKPAPASAVSTAVPQ

SEQ ID NO: 48 - protein, 24 aa, Escherichia coli
VYNIQDETGQFKPAPASASTAVPQ

SEQ ID NO: 49 - protein, 25 aa, Escherichia coli
VYNIQDETGQFKPAPASGFSTAVPQ

SEQ ID NO: 50 - protein, 25 aa, Escherichia coli
VYNIQDETGQFKPAPASGASTAVPQ

SEQ ID NO: 51 - protein, 25 aa, Escherichia coli
VYNIQDETGQFKPAPASGGSTAVPQ

SEQ ID NO: 52 - protein, 25 aa, Escherichia coli
VYNIQDETGQFKPAPASGVSTAVPQ

SEQ ID NO: 53 - protein, 24 aa, Escherichia coli
VYNIQDETGQFKPAPASGSTAVPQ

SEQ ID NO: 54 - protein, 25 aa, Escherichia coli
VYNIQDETGQFKPAPASVFSTAVPQ

SEQ ID NO: 55 - protein, 25 aa, Escherichia coli
VYNIQDETGQFKPAPASVASTAVPQ

SEQ ID NO: 56 - protein, 25 aa, Escherichia coli
VYNIQDETGQFKPAPASVGSTAVPQ

SEQ ID NO: 57 - protein, 25 aa, Escherichia coli
VYNIQDETGQFKPAPASVVSTAVPQ

SEQ ID NO: 58 - protein, 24 aa, Escherichia coli
VYNIQDETGQFKPAPASVSTAVPQ

SEQ ID NO: 59 - protein, 25 aa, Escherichia coli
VYNIQDETGQFKPAPASSFSTAVPQ

SEQ ID NO: 60 - protein, 25 aa, Escherichia coli
VYNIQDETGQFKPAPASSASTAVPQ

SEQ ID NO: 61 - protein, 25 aa, Escherichia coli
VYNIQDETGQFKPAPASSGSTAVPQ

SEQ ID NO: 62 - protein, 25 aa, Escherichia coli
VYNIQDETGQFKPAPASSVSTAVPQ

SEQ ID NO: 63 - protein, 24 aa, Escherichia coli
VYNIQDETGQFKPAPASSSTAVPQ

SEQ ID NO: 64 - protein, 25 aa, Escherichia coli
VYNIQDETGQFKPAPASTFSTAVPQ

SEQ ID NO: 65 - protein, 25 aa, Escherichia coli
VYNIQDETGQFKPAPASTASTAVPQ

SEQ ID NO: 66 - protein, 25 aa, Escherichia coli
VYNIQDETGQFKPAPASTGSTAVPQ

SEQ ID NO: 67 - protein, 25 aa, Escherichia coli
VYNIQDETGQFKPAPASTVSTAVPQ

SEQ ID NO: 68 - protein, 24 aa, Escherichia coli
VYNIQDETGQFKPAPASTSTAVPQ

SEQ ID NO: 69 - protein, 24 aa, Escherichia coli
VYNIQDETGQFKPAPASFSTAVPQ

SEQ ID NO: 70 - protein, 24 aa, Escherichia coli
VYNIQDETGQFKPAPASASTAVPQ

SEQ ID NO: 71 - protein, 24 aa, Escherichia coli
VYNIQDETGQFKPAPASGSTAVPQ

SEQ ID NO: 72 - protein, 24 aa, Escherichia coli
VYNIQDETGQFKPAPASVSTAVPQ

SEQ ID NO: 73 - protein, 23 aa, Escherichia coli
VYNIQDETGQFKPAPASSTAVPQ

SEQ ID NO: 74 - protein, 25 aa, Escherichia coli
VYNIQDETGQFKPGPASNFSTAVPQ

SEQ ID NO: 75 - protein, 25 aa, Escherichia coli
VYNIQDETGQFKPGPASNASTAVPQ

SEQ ID NO: 76 - protein, 25 aa, Escherichia coli
VYNIQDETGQFKPGPASNGSTAVPQ

SEQ ID NO: 77 - protein, 25 aa, Escherichia coli
VYNIQDETGQFKPGPASNVSTAVPQ

SEQ ID NO: 78 - protein, 24 aa, Escherichia coli
VYNIQDETGQFKPGPASNSTAVPQ

SEQ ID NO: 79 - protein, 25 aa, Escherichia coli
VYNIQDETGQFKPGPASAFSTAVPQ

SEQ ID NO: 80 - protein, 25 aa, Escherichia coli
VYNIQDETGQFKPGPASAASTAVPQ

SEQ ID NO: 81 - protein, 25 aa, Escherichia coli
VYNIQDETGQFKPGPASAGSTAVPQ

SEQ ID NO: 82 - protein, 25 aa, Escherichia coli
VYNIQDETGQFKPGPASAVSTAVPQ

SEQ ID NO: 83 - protein, 24 aa, Escherichia coli
VYNIQDETGQFKPGPASASTAVPQ

SEQ ID NO: 84 - protein, 25 aa, Escherichia coli
VYNIQDETGQFKPGPASGFSTAVPQ

SEQ ID NO: 85 - protein, 25 aa, Escherichia coli
VYNIQDETGQFKPGPASGASTAVPQ

SEQ ID NO: 86 - protein, 25 aa, Escherichia coli
VYNIQDETGQFKPGPASGGSTAVPQ

SEQ ID NO: 87 - protein, 25 aa, Escherichia coli
VYNIQDETGQFKPGPASGVSTAVPQ

SEQ ID NO: 88 - protein, 24 aa, Escherichia coli
VYNIQDETGQFKPGPASGSTAVPQ

SEQ ID NO: 89 - protein, 25 aa, Escherichia coli
VYNIQDETGQFKPGPASVFSTAVPQ

SEQ ID NO: 90 - protein, 25 aa, Escherichia coli
VYNIQDETGQFKPGPASVASTAVPQ

SEQ ID NO: 91 - protein, 25 aa, Escherichia coli
VYNIQDETGQFKPGPASVGSTAVPQ

SEQ ID NO: 92 - protein, 25 aa, Escherichia coli
VYNIQDETGQFKPGPASVVSTAVPQ

SEQ ID NO: 93 - protein, 24 aa, Escherichia coli
VYNIQDETGQFKPGPASVSTAVPQ

SEQ ID NO: 94 - protein, 25 aa, Escherichia coli
VYNIQDETGQFKPGPASSFSTAVPQ

SEQ ID NO: 95 - protein, 25 aa, Escherichia coli
VYNIQDETGQFKPGPASSASTAVPQ

SEQ ID NO: 96 - protein, 25 aa, Escherichia coli
VYNIQDETGQFKPGPASSGSTAVPQ

SEQ ID NO: 97 - protein, 25 aa, Escherichia coli
VYNIQDETGQFKPGPASSVSTAVPQ

SEQ ID NO: 98 - protein, 24 aa, Escherichia coli
VYNIQDETGQFKPGPASSSTAVPQ

SEQ ID NO: 99 - protein, 25 aa, Escherichia coli
VYNIQDETGQFKPGPASTFSTAVPQ

SEQ ID NO: 100 - protein, 25 aa, Escherichia coli
VYNIQDETGQFKPGPASTASTAVPQ

SEQ ID NO: 101 - protein, 25 aa, Escherichia coli
VYNIQDETGQFKPGPASTGSTAVPQ

SEQ ID NO: 102 - protein, 25 aa, Escherichia coli
VYNIQDETGQFKPGPASTVSTAVPQ

SEQ ID NO: 103 - protein, 24 aa, Escherichia coli
VYNIQDETGQFKPGPASTSTAVPQ

SEQ ID NO: 104 - protein, 24 aa, Escherichia coli
VYNIQDETGQFKPGPASFSTAVPQ

SEQ ID NO: 105 - protein, 24 aa, Escherichia coli
VYNIQDETGQFKPGPASASTAVPQ

SEQ ID NO: 106 - protein, 24 aa, Escherichia coli
VYNIQDETGQFKPGPASGSTAVPQ

SEQ ID NO: 107 - protein, 24 aa, Escherichia coli
VYNIQDETGQFKPGPASVSTAVPQ

SEQ ID NO: 108 - protein, 23 aa, Escherichia coli
VYNIQDETGQFKPGPASSTAVPQ

SEQ ID NO: 109 - protein, 25 aa, Escherichia coli
VYNIQDETGQFKPVPASNFSTAVPQ

SEQ ID NO: 110 - protein, 25 aa, Escherichia coli
VYNIQDETGQFKPVPASNASTAVPQ

SEQ ID NO: 111 - protein, 25 aa, Escherichia coli
VYNIQDETGQFKPVPASNGSTAVPQ

SEQ ID NO: 112 - protein, 25 aa, Escherichia coli
VYNIQDETGQFKPVPASNVSTAVPQ

SEQ ID NO: 113 - protein, 24 aa, Escherichia coli
VYNIQDETGQFKPVPASNSTAVPQ

SEQ ID NO: 114 - protein, 25 aa, Escherichia coli
VYNIQDETGQFKPVPASAFSTAVPQ

SEQ ID NO: 115 - protein, 25 aa, Escherichia coli
VYNIQDETGQFKPVPASAASTAVPQ

SEQ ID NO: 116 - protein, 25 aa, Escherichia coli
VYNIQDETGQFKPVPASAGSTAVPQ

SEQ ID NO: 117 - protein, 25 aa, Escherichia coli
VYNIQDETGQFKPVPASAVSTAVPQ

SEQ ID NO: 118 - protein, 24 aa, Escherichia coli
VYNIQDETGQFKPVPASASTAVPQ

SEQ ID NO: 119 - protein, 25 aa, Escherichia coli
VYNIQDETGQFKPVPASGFSTAVPQ

SEQ ID NO: 120 - protein, 25 aa, Escherichia coli
VYNIQDETGQFKPVPASGASTAVPQ

SEQ ID NO: 121 - protein, 25 aa, Escherichia coli
VYNIQDETGQFKPVPASGGSTAVPQ

SEQ ID NO: 122 - protein, 25 aa, Escherichia coli
VYNIQDETGQFKPVPASGVSTAVPQ

SEQ ID NO: 123 - protein, 24 aa, Escherichia coli
VYNIQDETGQFKPVPASGSTAVPQ

SEQ ID NO: 124 - protein, 25 aa, Escherichia coli
VYNIQDETGQFKPVPASVFSTAVPQ

SEQ ID NO: 125 - protein, 25 aa, Escherichia coli
VYNIQDETGQFKPVPASVASTAVPQ

SEQ ID NO: 126 - protein, 25 aa, Escherichia coli
VYNIQDETGQFKPVPASVGSTAVPQ

SEQ ID NO: 127 - protein, 25 aa, Escherichia coli
VYNIQDETGQFKPVPASVVSTAVPQ

SEQ ID NO: 128 - protein, 24 aa, Escherichia coli
VYNIQDETGQFKPVPASVSTAVPQ

SEQ ID NO: 129 - protein, 25 aa, Escherichia coli
VYNIQDETGQFKPVPASSFSTAVPQ

SEQ ID NO: 130 - protein, 25 aa, Escherichia coli
VYNIQDETGQFKPVPASSASTAVPQ

SEQ ID NO: 131 - protein, 25 aa, Escherichia coli
VYNIQDETGQFKPVPASSGSTAVPQ

SEQ ID NO: 132 - protein, 25 aa, Escherichia coli
VYNIQDETGQFKPVPASSVSTAVPQ

SEQ ID NO: 133 - protein, 24 aa, Escherichia coli
VYNIQDETGQFKPVPASSSTAVPQ

SEQ ID NO: 134 - protein, 25 aa, Escherichia coli
VYNIQDETGQFKPVPASTFSTAVPQ

SEQ ID NO: 135 - protein, 25 aa, Escherichia coli
VYNIQDETGQFKPVPASTASTAVPQ

SEQ ID NO: 136 - protein, 25 aa, Escherichia coli
VYNIQDETGQFKPVPASTGSTAVPQ

SEQ ID NO: 137 - protein, 25 aa, Escherichia coli
VYNIQDETGQFKPVPASTVSTAVPQ

SEQ ID NO: 138 - protein, 24 aa, Escherichia coli
VYNIQDETGQFKPVPASTSTAVPQ

SEQ ID NO: 139 - protein, 24 aa, Escherichia coli
VYNIQDETGQFKPVPASFSTAVPQ

SEQ ID NO: 140 - protein, 24 aa, Escherichia coli
VYNIQDETGQFKPVPASASTAVPQ

SEQ ID NO: 141 - protein, 24 aa, Escherichia coli
VYNIQDETGQFKPVPASGSTAVPQ

SEQ ID NO: 142 - protein, 24 aa, Escherichia coli
VYNIQDETGQFKPVPASVSTAVPQ

SEQ ID NO: 143 - protein, 23 aa, Escherichia coli
VYNIQDETGQFKPVPASSTAVPQ

SEQ ID NO: 144 - protein, 25 aa, Escherichia coli
VYNIQDETGQFKPLPASNFSTAVPQ

SEQ ID NO: 145 - protein, 25 aa, Escherichia coli
VYNIQDETGQFKPLPASNASTAVPQ

SEQ ID NO: 146 - protein, 25 aa, Escherichia coli
VYNIQDETGQFKPLPASNGSTAVPQ

SEQ ID NO: 147 - protein, 25 aa, Escherichia coli
VYNIQDETGQFKPLPASNVSTAVPQ

SEQ ID NO: 148 - protein, 24 aa, Escherichia coli
VYNIQDETGQFKPLPASNSTAVPQ

SEQ ID NO: 149 - protein, 25 aa, Escherichia coli
VYNIQDETGQFKPLPASAFSTAVPQ

SEQ ID NO: 150 - protein, 25 aa, Escherichia coli
VYNIQDETGQFKPLPASAASTAVPQ

SEQ ID NO: 151 - protein, 25 aa, Escherichia coli
VYNIQDETGQFKPLPASAGSTAVPQ

SEQ ID NO: 152 - protein, 25 aa, Escherichia coli
VYNIQDETGQFKPLPASAVSTAVPQ

SEQ ID NO: 153 - protein, 24 aa, Escherichia coli
VYNIQDETGQFKPLPASASTAVPQ

SEQ ID NO: 154 - protein, 25 aa, Escherichia coli
VYNIQDETGQFKPLPASGFSTAVPQ

SEQ ID NO: 155 - protein, 25 aa, Escherichia coli
VYNIQDETGQFKPLPASGASTAVPQ

SEQ ID NO: 156 - protein, 25 aa, Escherichia coli
VYNIQDETGQFKPLPASGGSTAVPQ

SEQ ID NO: 157 - protein, 25 aa, Escherichia coli
VYNIQDETGQFKPLPASGVSTAVPQ

SEQ ID NO: 158 - protein, 24 aa, Escherichia coli
VYNIQDETGQFKPLPASGSTAVPQ

SEQ ID NO: 159 - protein, 25 aa, Escherichia coli
VYNIQDETGQFKPLPASVFSTAVPQ

SEQ ID NO: 160 - protein, 25 aa, Escherichia coli
VYNIQDETGQFKPLPASVASTAVPQ

SEQ ID NO: 161 - protein, 25 aa, Escherichia coli
VYNIQDETGQFKPLPASVGSTAVPQ

SEQ ID NO: 162 - protein, 25 aa, Escherichia coli
VYNIQDETGQFKPLPASVVSTAVPQ

SEQ ID NO: 163 - protein, 24 aa, Escherichia coli
VYNIQDETGQFKPLPASVSTAVPQ

SEQ ID NO: 164 - protein, 25 aa, Escherichia coli
VYNIQDETGQFKPLPASSFSTAVPQ

SEQ ID NO: 165 - protein, 25 aa, Escherichia coli
VYNIQDETGQFKPLPASSASTAVPQ

SEQ ID NO: 166 - protein, 25 aa, Escherichia coli
VYNIQDETGQFKPLPASSGSTAVPQ

SEQ ID NO: 167 - protein, 25 aa, Escherichia coli
VYNIQDETGQFKPLPASSVSTAVPQ

SEQ ID NO: 168 - protein, 24 aa, Escherichia coli
VYNIQDETGQFKPLPASSSTAVPQ

SEQ ID NO: 169 - protein, 25 aa, Escherichia coli
VYNIQDETGQFKPLPASTFSTAVPQ

SEQ ID NO: 170 - protein, 25 aa, Escherichia coli
VYNIQDETGQFKPLPASTASTAVPQ

SEQ ID NO: 171 - protein, 25 aa, Escherichia coli
VYNIQDETGQFKPLPASTGSTAVPQ

SEQ ID NO: 172 - protein, 25 aa, Escherichia coli
VYNIQDETGQFKPLPASTVSTAVPQ

SEQ ID NO: 173 - protein, 24 aa, Escherichia coli
VYNIQDETGQFKPLPASTSTAVPQ

SEQ ID NO: 174 - protein, 24 aa, Escherichia coli
VYNIQDETGQFKPLPASFSTAVPQ

SEQ ID NO: 175 - protein, 24 aa, Escherichia coli
VYNIQDETGQFKPLPASASTAVPQ

SEQ ID NO: 176 - protein, 24 aa, Escherichia coli
VYNIQDETGQFKPLPASGSTAVPQ

SEQ ID NO: 177 - protein, 24 aa, Escherichia coli
VYNIQDETGQFKPLPASVSTAVPQ

SEQ ID NO: 178 - protein, 23 aa, Escherichia coli
VYNIQDETGQFKPLPASSTAVPQ

SEQ ID NO: 179 - protein, 25 aa, Escherichia coli
VYNIQDETGQFKPIPASNFSTAVPQ

SEQ ID NO: 180 - protein, 25 aa, Escherichia coli
VYNIQDETGQFKPIPASNASTAVPQ

SEQ ID NO: 181 - protein, 25 aa, Escherichia coli
VYNIQDETGQFKPIPASNGSTAVPQ

SEQ ID NO: 182 - protein, 25 aa, Escherichia coli
VYNIQDETGQFKPIPASNVSTAVPQ

SEQ ID NO: 183 - protein, 24 aa, Escherichia coli
VYNIQDETGQFKPIPASNSTAVPQ

SEQ ID NO: 184 - protein, 25 aa, Escherichia coli
VYNIQDETGQFKPIPASAFSTAVPQ

SEQ ID NO: 185 - protein, 25 aa, Escherichia coli
VYNIQDETGQFKPIPASAASTAVPQ

SEQ ID NO: 186 - protein, 25 aa, Escherichia coli
VYNIQDETGQFKPIPASAGSTAVPQ

SEQ ID NO: 187 - protein, 25 aa, Escherichia coli
VYNIQDETGQFKPIPASAVSTAVPQ

SEQ ID NO: 188 - protein, 24 aa, Escherichia coli
VYNIQDETGQFKPIPASASTAVPQ

SEQ ID NO: 189 - protein, 25 aa, Escherichia coli
VYNIQDETGQFKPIPASGFSTAVPQ

SEQ ID NO: 190 - protein, 25 aa, Escherichia coli
VYNIQDETGQFKPIPASGASTAVPQ

SEQ ID NO: 191 - protein, 25 aa, Escherichia coli
VYNIQDETGQFKPIPASGGSTAVPQ

SEQ ID NO: 192 - protein, 25 aa, Escherichia coli
VYNIQDETGQFKPIPASGVSTAVPQ

SEQ ID NO: 193 - protein, 24 aa, Escherichia coli
VYNIQDETGQFKPIPASGSTAVPQ

SEQ ID NO: 194 - protein, 25 aa, Escherichia coli
VYNIQDETGQFKPIPASVFSTAVPQ

SEQ ID NO: 195 - protein, 25 aa, Escherichia coli
VYNIQDETGQFKPIPASVASTAVPQ

SEQ ID NO: 196 - protein, 25 aa, Escherichia coli
VYNIQDETGQFKPIPASVGSTAVPQ

SEQ ID NO: 197 - protein, 25 aa, Escherichia coli
VYNIQDETGQFKPIPASVVSTAVPQ

SEQ ID NO: 198 - protein, 24 aa, Escherichia coli
VYNIQDETGQFKPIPASVSTAVPQ

SEQ ID NO: 199 - protein, 25 aa, Escherichia coli
VYNIQDETGQFKPIPASSFSTAVPQ

SEQ ID NO: 200 - protein, 25 aa, Escherichia coli
VYNIQDETGQFKPIPASSASTAVPQ

SEQ ID NO: 201 - protein, 25 aa, Escherichia coli
VYNIQDETGQFKPIPASSGSTAVPQ

SEQ ID NO: 202 - protein, 25 aa, Escherichia coli
VYNIQDETGQFKPIPASSVSTAVPQ

SEQ ID NO: 203 - protein, 24 aa, Escherichia coli
VYNIQDETGQFKPIPASSSTAVPQ

SEQ ID NO: 204 - protein, 25 aa, Escherichia coli
VYNIQDETGQFKPIPASTFSTAVPQ

SEQ ID NO: 205 - protein, 25 aa, Escherichia coli
VYNIQDETGQFKPIPASTASTAVPQ

SEQ ID NO: 206 - protein, 25 aa, Escherichia coli
VYNIQDETGQFKPIPASTGSTAVPQ

SEQ ID NO: 207 - protein, 25 aa, Escherichia coli
VYNIQDETGQFKPIPASTVSTAVPQ

SEQ ID NO: 208 - protein, 24 aa, Escherichia coli
VYNIQDETGQFKPIPASTSTAVPQ

SEQ ID NO: 209 - protein, 24 aa, Escherichia coli
VYNIQDETGQFKPIPASFSTAVPQ

SEQ ID NO: 210 - protein, 24 aa, Escherichia coli
VYNIQDETGQFKPIPASASTAVPQ

SEQ ID NO: 211 - protein, 24 aa, Escherichia coli
VYNIQDETGQFKPIPASGSTAVPQ

SEQ ID NO: 212 - protein, 24 aa, Escherichia coli
VYNIQDETGQFKPIPASVSTAVPQ

SEQ ID NO: 213 - protein, 23 aa, Escherichia coli
VYNIQDETGQFKPIPASSTAVPQ

SEQ ID NO: 214 - protein, 25 aa, Escherichia coli
VYNIQDETGQFKPNPASNFSTAVPQ

SEQ ID NO: 215 - protein, 25 aa, Escherichia coli
VYNIQDETGQFKPNPASNASTAVPQ

SEQ ID NO: 216 - protein, 25 aa, Escherichia coli
VYNIQDETGQFKPNPASNGSTAVPQ

SEQ ID NO: 217 - protein, 25 aa, Escherichia coli
VYNIQDETGQFKPNPASNVSTAVPQ

SEQ ID NO: 218 - protein, 24 aa, Escherichia coli
VYNIQDETGQFKPNPASNSTAVPQ

SEQ ID NO: 219 - protein, 25 aa, Escherichia coli
VYNIQDETGQFKPNPASAFSTAVPQ

SEQ ID NO: 220 - protein, 25 aa, Escherichia coli
VYNIQDETGQFKPNPASAASTAVPQ

SEQ ID NO: 221 - protein, 25 aa, Escherichia coli
VYNIQDETGQFKPNPASAGSTAVPQ

SEQ ID NO: 222 - protein, 25 aa, Escherichia coli
VYNIQDETGQFKPNPASAVSTAVPQ

SEQ ID NO: 223 - protein, 24 aa, Escherichia coli
VYNIQDETGQFKPNPASASTAVPQ

SEQ ID NO: 224 - protein, 25 aa, Escherichia coli
VYNIQDETGQFKPNPASGFSTAVPQ

SEQ ID NO: 225 - protein, 25 aa, Escherichia coli
VYNIQDETGQFKPNPASGASTAVPQ

SEQ ID NO: 226 - protein, 25 aa, Escherichia coli
VYNIQDETGQFKPNPASGGSTAVPQ

SEQ ID NO: 227 - protein, 25 aa, Escherichia coli
VYNIQDETGQFKPNPASGVSTAVPQ

SEQ ID NO: 228 - protein, 24 aa, Escherichia coli
VYNIQDETGQFKPNPASGSTAVPQ

SEQ ID NO: 229 - protein, 25 aa, Escherichia coli
VYNIQDETGQFKPNPASVFSTAVPQ

SEQ ID NO: 230 - protein, 25 aa, Escherichia coli
VYNIQDETGQFKPNPASVASTAVPQ

SEQ ID NO: 231 - protein, 25 aa, Escherichia coli
VYNIQDETGQFKPNPASVGSTAVPQ

SEQ ID NO: 232 - protein, 25 aa, Escherichia coli
VYNIQDETGQFKPNPASVVSTAVPQ

SEQ ID NO: 233 - protein, 24 aa, Escherichia coli
VYNIQDETGQFKPNPASVSTAVPQ

SEQ ID NO: 234 - protein, 25 aa, Escherichia coli
VYNIQDETGQFKPNPASSFSTAVPQ

SEQ ID NO: 235 - protein, 25 aa, Escherichia coli
VYNIQDETGQFKPNPASSASTAVPQ

SEQ ID NO: 236 - protein, 25 aa, Escherichia coli
VYNIQDETGQFKPNPASSGSTAVPQ

SEQ ID NO: 237 - protein, 25 aa, Escherichia coli
VYNIQDETGQFKPNPASSVSTAVPQ

SEQ ID NO: 238 - protein, 24 aa, Escherichia coli
VYNIQDETGQFKPNPASSSTAVPQ

SEQ ID NO: 239 - protein, 25 aa, Escherichia coli
VYNIQDETGQFKPNPASTFSTAVPQ

SEQ ID NO: 240 - protein, 25 aa, Escherichia coli
VYNIQDETGQFKPNPASTASTAVPQ

SEQ ID NO: 241 - protein, 25 aa, Escherichia coli
VYNIQDETGQFKPNPASTGSTAVPQ

SEQ ID NO: 242 - protein, 25 aa, Escherichia coli
VYNIQDETGQFKPNPASTVSTAVPQ

SEQ ID NO: 243 - protein, 24 aa, Escherichia coli
VYNIQDETGQFKPNPASTSTAVPQ

SEQ ID NO: 244 - protein, 24 aa, Escherichia coli
VYNIQDETGQFKPNPASFSTAVPQ

SEQ ID NO: 245 - protein, 24 aa, Escherichia coli
VYNIQDETGQFKPNPASASTAVPQ

SEQ ID NO: 246 - protein, 24 aa, Escherichia coli
VYNIQDETGQFKPNPASGSTAVPQ

SEQ ID NO: 247 - protein, 24 aa, Escherichia coli
VYNIQDETGQFKPNPASVSTAVPQ

SEQ ID NO: 248 - protein, 23 aa, Escherichia coli
VYNIQDETGQFKPNPASSTAVPQ

SEQ ID NO: 249 - protein, 25 aa, Escherichia coli
VYNIQDETGQFKPQPASNFSTAVPQ

SEQ ID NO: 250 - protein, 25 aa, Escherichia coli
VYNIQDETGQFKPQPASNASTAVPQ

SEQ ID NO: 251 - protein, 25 aa, Escherichia coli
VYNIQDETGQFKPQPASNGSTAVPQ

SEQ ID NO: 252 - protein, 25 aa, Escherichia coli
VYNIQDETGQFKPQPASNVSTAVPQ

SEQ ID NO: 253 - protein, 24 aa, Escherichia coli
VYNIQDETGQFKPQPASNSTAVPQ

SEQ ID NO: 254 - protein, 25 aa, Escherichia coli
VYNIQDETGQFKPQPASAFSTAVPQ

SEQ ID NO: 255 - protein, 25 aa, Escherichia coli
VYNIQDETGQFKPQPASAASTAVPQ

SEQ ID NO: 256 - protein, 25 aa, Escherichia coli
VYNIQDETGQFKPQPASAGSTAVPQ

SEQ ID NO: 257 - protein, 25 aa, Escherichia coli
VYNIQDETGQFKPQPASAVSTAVPQ

SEQ ID NO: 258 - protein, 24 aa, Escherichia coli
VYNIQDETGQFKPQPASASTAVPQ

SEQ ID NO: 259 - protein, 25 aa, Escherichia coli
VYNIQDETGQFKPQPASGFSTAVPQ

SEQ ID NO: 260 - protein, 25 aa, Escherichia coli
VYNIQDETGQFKPQPASGASTAVPQ

SEQ ID NO: 261 - protein, 25 aa, Escherichia coli
VYNIQDETGQFKPQPASGGSTAVPQ

SEQ ID NO: 262 - protein, 25 aa, Escherichia coli
VYNIQDETGQFKPQPASGVSTAVPQ

SEQ ID NO: 263 - protein, 24 aa, Escherichia coli
VYNIQDETGQFKPQPASGSTAVPQ

SEQ ID NO: 264 - protein, 25 aa, Escherichia coli
VYNIQDETGQFKPQPASVFSTAVPQ

SEQ ID NO: 265 - protein, 25 aa, Escherichia coli
VYNIQDETGQFKPQPASVASTAVPQ

SEQ ID NO: 266 - protein, 25 aa, Escherichia coli
VYNIQDETGQFKPQPASVGSTAVPQ

SEQ ID NO: 267 - protein, 25 aa, Escherichia coli
VYNIQDETGQFKPQPASVVSTAVPQ

SEQ ID NO: 268 - protein, 24 aa, Escherichia coli
VYNIQDETGQFKPQPASVSTAVPQ

SEQ ID NO: 269 - protein, 25 aa, Escherichia coli
VYNIQDETGQFKPQPASSFSTAVPQ

SEQ ID NO: 270 - protein, 25 aa, Escherichia coli
VYNIQDETGQFKPQPASSASTAVPQ

SEQ ID NO: 271 - protein, 25 aa, Escherichia coli
VYNIQDETGQFKPQPASSGSTAVPQ

SEQ ID NO: 272 - protein, 25 aa, Escherichia coli
VYNIQDETGQFKPQPASSVSTAVPQ

SEQ ID NO: 273 - protein, 24 aa, Escherichia coli
VYNIQDETGQFKPQPASSSTAVPQ

SEQ ID NO: 274 - protein, 25 aa, Escherichia coli
VYNIQDETGQFKPQPASTFSTAVPQ

SEQ ID NO: 275 - protein, 25 aa, Escherichia coli
VYNIQDETGQFKPQPASTASTAVPQ

SEQ ID NO: 276 - protein, 25 aa, Escherichia coli
VYNIQDETGQFKPQPASTGSTAVPQ

SEQ ID NO: 277 - protein, 25 aa, Escherichia coli
VYNIQDETGQFKPQPASTVSTAVPQ

SEQ ID NO: 278 - protein, 24 aa, Escherichia coli
VYNIQDETGQFKPQPASTSTAVPQ

SEQ ID NO: 279 - protein, 24 aa, Escherichia coli
VYNIQDETGQFKPQPASFSTAVPQ

SEQ ID NO: 280 - protein, 24 aa, Escherichia coli
VYNIQDETGQFKPQPASASTAVPQ

SEQ ID NO: 281 - protein, 24 aa, Escherichia coli
VYNIQDETGQFKPQPASGSTAVPQ

SEQ ID NO: 282 - protein, 24 aa, Escherichia coli
VYNIQDETGQFKPQPASVSTAVPQ

SEQ ID NO: 283 - protein, 23 aa, Escherichia coli
VYNIQDETGQFKPQPASSTAVPQ

SEQ ID NO: 284 - protein, 25 aa, Escherichia coli
VYNIQDETGQFKPFPASNFSTAVPQ

SEQ ID NO: 285 - protein, 25 aa, Escherichia coli
VYNIQDETGQFKPFPASNASTAVPQ

SEQ ID NO: 286 - protein, 25 aa, Escherichia coli
VYNIQDETGQFKPFPASNGSTAVPQ

SEQ ID NO: 287 - protein, 25 aa, Escherichia coli
VYNIQDETGQFKPFPASNVSTAVPQ

SEQ ID NO: 288 - protein, 24 aa, Escherichia coli
VYNIQDETGQFKPFPASNSTAVPQ

SEQ ID NO: 289 - protein, 25 aa, Escherichia coli
VYNIQDETGQFKPFPASAFSTAVPQ

SEQ ID NO: 290 - protein, 25 aa, Escherichia coli
VYNIQDETGQFKPFPASAASTAVPQ

SEQ ID NO: 291 - protein, 25 aa, Escherichia coli
VYNIQDETGQFKPFPASAGSTAVPQ

SEQ ID NO: 292 - protein, 25 aa, Escherichia coli
VYNIQDETGQFKPFPASAVSTAVPQ

SEQ ID NO: 293 - protein, 24 aa, Escherichia coli
VYNIQDETGQFKPFPASASTAVPQ

SEQ ID NO: 294 - protein, 25 aa, Escherichia coli
VYNIQDETGQFKPFPASGFSTAVPQ

SEQ ID NO: 295 - protein, 25 aa, Escherichia coli
VYNIQDETGQFKPFPASGASTAVPQ

SEQ ID NO: 296 - protein, 25 aa, Escherichia coli
VYNIQDETGQFKPFPASGGSTAVPQ

SEQ ID NO: 297 - protein, 25 aa, Escherichia coli
VYNIQDETGQFKPFPASGVSTAVPQ

SEQ ID NO: 298 - protein, 24 aa, Escherichia coli
VYNIQDETGQFKPFPASGSTAVPQ

SEQ ID NO: 299 - protein, 25 aa, Escherichia coli
VYNIQDETGQFKPFPASVFSTAVPQ

SEQ ID NO: 300 - protein, 25 aa, Escherichia coli
VYNIQDETGQFKPFPASVASTAVPQ

SEQ ID NO: 301 - protein, 25 aa, Escherichia coli
VYNIQDETGQFKPFPASVGSTAVPQ

SEQ ID NO: 302 - protein, 25 aa, Escherichia coli
VYNIQDETGQFKPFPASVVSTAVPQ

SEQ ID NO: 303 - protein, 24 aa, Escherichia coli
VYNIQDETGQFKPFPASVSTAVPQ

SEQ ID NO: 304 - protein, 25 aa, Escherichia coli
VYNIQDETGQFKPFPASSFSTAVPQ

SEQ ID NO: 305 - protein, 25 aa, Escherichia coli
VYNIQDETGQFKPFPASSASTAVPQ

SEQ ID NO: 306 - protein, 25 aa, Escherichia coli
VYNIQDETGQFKPFPASSGSTAVPQ

SEQ ID NO: 307 - protein, 25 aa, Escherichia coli
VYNIQDETGQFKPFPASSVSTAVPQ

SEQ ID NO: 308 - protein, 24 aa, Escherichia coli
VYNIQDETGQFKPFPASSSTAVPQ

SEQ ID NO: 309 - protein, 25 aa, Escherichia coli
VYNIQDETGQFKPFPASTFSTAVPQ

SEQ ID NO: 310 - protein, 25 aa, Escherichia coli
VYNIQDETGQFKPFPASTASTAVPQ

SEQ ID NO: 311 - protein, 25 aa, Escherichia coli
VYNIQDETGQFKPFPASTGSTAVPQ

SEQ ID NO: 312 - protein, 25 aa, Escherichia coli
VYNIQDETGQFKPFPASTVSTAVPQ

SEQ ID NO: 313 - protein, 24 aa, Escherichia coli
VYNIQDETGQFKPFPASTSTAVPQ

SEQ ID NO: 314 - protein, 24 aa, Escherichia coli
VYNIQDETGQFKPFPASFSTAVPQ

SEQ ID NO: 315 - protein, 24 aa, Escherichia coli
VYNIQDETGQFKPFPASASTAVPQ

SEQ ID NO: 316 - protein, 24 aa, Escherichia coli
VYNIQDETGQFKPFPASGSTAVPQ

SEQ ID NO: 317 - protein, 24 aa, Escherichia coli
VYNIQDETGQFKPFPASVSTAVPQ

SEQ ID NO: 318 - protein, 23 aa, Escherichia coli
VYNIQDETGQFKPFPASSTAVPQ

SEQ ID NO: 319 - protein, 24 aa, Escherichia coli
VYNIQDETGQFKPPASNFSTAVPQ

SEQ ID NO: 320 - protein, 24 aa, Escherichia coli
VYNIQDETGQFKPPASNASTAVPQ

SEQ ID NO: 321 - protein, 24 aa, Escherichia coli
VYNIQDETGQFKPPASNGSTAVPQ

SEQ ID NO: 322 - protein, 24 aa, Escherichia coli
VYNIQDETGQFKPPASNVSTAVPQ

SEQ ID NO: 323 - protein, 23 aa, Escherichia coli
VYNIQDETGQFKPPASNSTAVPQ

SEQ ID NO: 324 - protein, 24 aa, Escherichia coli
VYNIQDETGQFKPPASAFSTAVPQ

SEQ ID NO: 325 - protein, 24 aa, Escherichia coli
VYNIQDETGQFKPPASAASTAVPQ

SEQ ID NO: 326 - protein, 24 aa, Escherichia coli
VYNIQDETGQFKPPASAGSTAVPQ

SEQ ID NO: 327 - protein, 24 aa, Escherichia coli
VYNIQDETGQFKPPASAVSTAVPQ

SEQ ID NO: 328 - protein, 23 aa, Escherichia coli
VYNIQDETGQFKPPASASTAVPQ

SEQ ID NO: 329 - protein, 24 aa, Escherichia coli
VYNIQDETGQFKPPASGFSTAVPQ

SEQ ID NO: 330 - protein, 24 aa, Escherichia coli
VYNIQDETGQFKPPASGASTAVPQ

SEQ ID NO: 331 - protein, 24 aa, Escherichia coli
VYNIQDETGQFKPPASGGSTAVPQ

SEQ ID NO: 332 - protein, 24 aa, Escherichia coli
VYNIQDETGQFKPPASGVSTAVPQ

SEQ ID NO: 333 - protein, 23 aa, Escherichia coli
VYNIQDETGQFKPPASGSTAVPQ

SEQ ID NO: 334 - protein, 24 aa, Escherichia coli
VYNIQDETGQFKPPASVFSTAVPQ

SEQ ID NO: 335 - protein, 24 aa, Escherichia coli
VYNIQDETGQFKPPASVASTAVPQ

SEQ ID NO: 336 - protein, 24 aa, Escherichia coli
VYNIQDETGQFKPPASVGSTAVPQ

SEQ ID NO: 337 - protein, 24 aa, Escherichia coli
VYNIQDETGQFKPPASVVSTAVPQ

SEQ ID NO: 338 - protein, 23 aa, Escherichia coli
VYNIQDETGQFKPPASVSTAVPQ

SEQ ID NO: 339 - protein, 24 aa, Escherichia coli
VYNIQDETGQFKPPASSFSTAVPQ

SEQ ID NO: 340 - protein, 24 aa, Escherichia coli
VYNIQDETGQFKPPASSASTAVPQ

SEQ ID NO: 341 - protein, 24 aa, Escherichia coli
VYNIQDETGQFKPPASSGSTAVPQ

SEQ ID NO: 342 - protein, 24 aa, Escherichia coli
VYNIQDETGQFKPPASSVSTAVPQ

SEQ ID NO: 343 - protein, 23 aa, Escherichia coli
VYNIQDETGQFKPPASSSTAVPQ

SEQ ID NO: 344 - protein, 24 aa, Escherichia coli
VYNIQDETGQFKPPASTFSTAVPQ

SEQ ID NO: 345 - protein, 24 aa, Escherichia coli
VYNIQDETGQFKPPASTASTAVPQ

SEQ ID NO: 346 - protein, 24 aa, Escherichia coli
VYNIQDETGQFKPPASTGSTAVPQ

SEQ ID NO: 347 - protein, 24 aa, Escherichia coli
VYNIQDETGQFKPPASTVSTAVPQ

SEQ ID NO: 348 - protein, 23 aa, Escherichia coli
VYNIQDETGQFKPPASTSTAVPQ

SEQ ID NO: 349 - protein, 23 aa, Escherichia coli
VYNIQDETGQFKPPASFSTAVPQ

SEQ ID NO: 350 - protein, 23 aa, Escherichia coli
VYNIQDETGQFKPPASASTAVPQ

SEQ ID NO: 351 - protein, 23 aa, Escherichia coli
VYNIQDETGQFKPPASGSTAVPQ

SEQ ID NO: 352 - protein, 23 aa, Escherichia coli
VYNIQDETGQFKPPASVSTAVPQ

SEQ ID NO: 353 - protein, 22 aa, Escherichia coli
VYNIQDETGQFKPPASSTAVPQ

SEQ ID NO: 354 - protein, 23 aa, Escherichia coli
VYNIQDETGQFKGGSNFSTAVPQ

SEQ ID NO: 355 - protein, 23 aa, Escherichia coli
VYNIQDETGQFKGGSNASTAVPQ

SEQ ID NO: 356 - protein, 23 aa, Escherichia coli
VYNIQDETGQFKGGSNGSTAVPQ

SEQ ID NO: 357 - protein, 23 aa, Escherichia coli
VYNIQDETGQFKGGSNVSTAVPQ

SEQ ID NO: 358 - protein, 22 aa, Escherichia coli
VYNIQDETGQFKGGSNSTAVPQ

SEQ ID NO: 359 - protein, 23 aa, Escherichia coli
VYNIQDETGQFKGGSAFSTAVPQ

SEQ ID NO: 360 - protein, 23 aa, Escherichia coli
VYNIQDETGQFKGGSAASTAVPQ

SEQ ID NO: 361 - protein, 23 aa, Escherichia coli
VYNIQDETGQFKGGSAGSTAVPQ

SEQ ID NO: 362 - protein, 23 aa, Escherichia coli
VYNIQDETGQFKGGSAVSTAVPQ

SEQ ID NO: 363 - protein, 22 aa, Escherichia coli
VYNIQDETGQFKGGSASTAVPQ

SEQ ID NO: 364 - protein, 23 aa, Escherichia coli
VYNIQDETGQFKGGSGFSTAVPQ

SEQ ID NO: 365 - protein, 23 aa, Escherichia coli
VYNIQDETGQFKGGSGASTAVPQ

SEQ ID NO: 366 - protein, 23 aa, Escherichia coli
VYNIQDETGQFKGGSGGSTAVPQ

SEQ ID NO: 367 - protein, 23 aa, Escherichia coli
VYNIQDETGQFKGGSGVSTAVPQ

SEQ ID NO: 368 - protein, 22 aa, Escherichia coli
VYNIQDETGQFKGGSGSTAVPQ

SEQ ID NO: 369 - protein, 23 aa, Escherichia coli
VYNIQDETGQFKGGSVFSTAVPQ

SEQ ID NO: 370 - protein, 23 aa, Escherichia coli
VYNIQDETGQFKGGSVASTAVPQ

SEQ ID NO: 371 - protein, 23 aa, Escherichia coli
VYNIQDETGQFKGGSVGSTAVPQ

SEQ ID NO: 372 - protein, 23 aa, Escherichia coli
VYNIQDETGQFKGGSVVSTAVPQ

SEQ ID NO: 373 - protein, 22 aa, Escherichia coli
VYNIQDETGQFKGGSVSTAVPQ

SEQ ID NO: 374 - protein, 23 aa, Escherichia coli
VYNIQDETGQFKGGSSFSTAVPQ

SEQ ID NO: 375 - protein, 23 aa, Escherichia coli
VYNIQDETGQFKGGSSASTAVPQ

SEQ ID NO: 376 - protein, 23 aa, Escherichia coli
VYNIQDETGQFKGGSSGSTAVPQ

SEQ ID NO: 377 - protein, 23 aa, Escherichia coli
VYNIQDETGQFKGGSSVSTAVPQ

SEQ ID NO: 378 - protein, 22 aa, Escherichia coli
VYNIQDETGQFKGGSSSTAVPQ

SEQ ID NO: 379 - protein, 23 aa, Escherichia coli
VYNIQDETGQFKGGSTFSTAVPQ

SEQ ID NO: 380 - protein, 23 aa, Escherichia coli
VYNIQDETGQFKGGSTASTAVPQ

SEQ ID NO: 381 - protein, 23 aa, Escherichia coli
VYNIQDETGQFKGGSTGSTAVPQ

SEQ ID NO: 382 - protein, 23 aa, Escherichia coli
VYNIQDETGQFKGGSTVSTAVPQ

SEQ ID NO: 383 - protein, 22 aa, Escherichia coli
VYNIQDETGQFKGGSTSTAVPQ

SEQ ID NO: 384 - protein, 22 aa, Escherichia coli
VYNIQDETGQFKGGSFSTAVPQ

SEQ ID NO: 385 - protein, 22 aa, Escherichia coli
VYNIQDETGQFKGGSASTAVPQ

SEQ ID NO: 386 - protein, 22 aa, Escherichia coli
VYNIQDETGQFKGGSGSTAVPQ

SEQ ID NO: 387 - protein, 22 aa, Escherichia coli
VYNIQDETGQFKGGSVSTAVPQ

SEQ ID NO: 388 - protein, 21 aa, Escherichia coli
VYNIQDETGQFKGGSSTAVPQ

SEQ ID NO: 389 - DNA, 786 bp, Escherichia coli
tgtctgaccgcaccgccgaaagaagcggcacgtccgaccctgatgccgcgtgcacagtcttataaagatctgacccatctgccggctccgacgggcaaaatttttgttagcgtctataacatccaggacgaaaccggtcaatttaaaccgtacccggcgagtaatttctccacggccgttccgcagagtgcaaccgctatgctggtcacggcactgaaagattcccgttggttcattccgctggaacgccagggcctgcaaaacctgctgaatgaacgtaaaattatccgcgcagctcaggaaaacggtaccgtggccattaacaatcgtattccgctgcaaagcctgaccgccgcaaacatcatggttgaaggctctatcatcggttacgaatcaaacgtcaaatcgggcggtgtgggcgcacgttattttggcattggtgctgatacccagtaccaactggaccagatcgcagttaacctgcgcgtggttaatgtcagcaccggcgaaattctgagctctgtgaataccagcaaaacgatcctgtcttacgaagtgcaggctggtgtttttcgtttcattgattatcaacgcctgctggaaggcgaagtcggttacacctcaaacgaaccggtgatgctgtgtctgatgtcggcgattgaaacgggtgttattttcctgatcaatgatggcatcgaccgtggtctgtgggatctgcagaacaaagccgaacgtcaaaatgacattctggtgaaataccgccacatgagtgttccgccggaatcc

SEQ ID NO: 390 - protein, 262 aa, Escherichia coli
CLTAPPKEAARPTLMPRAQSYKDLTHLPAPTGKIFVSVYNIQDETGQFKPYPASNFSTAVPQSATAMLVTALKDSRWFIPLERQGLQNLLNERKIIRAAQENGTVAINNRIPLQSLTAANIMVEGSIIGYESNVKSGGVGARYFGIGADTQYQLDQIAVNLRVVNVSTGEILSSVNTSKTILSYEVQAGVFRFIDYQRLLEGEVGYTSNEPVMLCLMSAIETGVIFLINDGIDRGLWDLQNKAERQNDILVKYRHMSVPPES

SEQ ID NO: 391 - protein, 248 aa, Citrobacter koseri
MPRAQSYKDLTHLPMPTGKIFVSVYNIQDETGQFKPYPASNFSTAVPQSATAMLVTALKDSRWFIPLERQGLQNLLNERKIIRAAQENGTVAINNRIPLQSLTAANIMVEGSIIGYESNVKSGGVGARYFGIGADTQYQLDQIAVNLRVVNVSTGEILSSVNTSKTILSYEVQAGVFRFIDYQRLLEGEIGYTSNEPVMLCLMSAIETGVIFLINDGIDRGLWDLQNKAERQNDILVKYRHMSVPPES

SEQ ID NO: 392 - protein, 223 aa, Salmonella enterica
CLTAPPKQAAKPTLMPRAQSYKDLTHLPAPTGKIFVSVYNIQDETGQFKPYPASNFSTAVPQSATAMLVTALKDSRWFIPLERQGLQNLLNERKIIRAAQENGTVAMNNRIPLQSLTAANIMVEGSIIGYESNVKSGGVGARYFGIGADTQYQLDQIAVNLRVVNVSTGEILSSVNTSKTILSYEVQAGVFRFIDYQRLLEGEIGYTSNEPVMLCLMSAIETG

SEQ ID NO: 393 - protein, 262 aa, Citrobacter amalonaticus
CLTAPPKEAAKPTLMPRAQSYKDLTHLPIPTGKIFVSVYNIQDETGQFKPYPASNFSTAVPQSATAMLVTALKDSRWFVPLERQGLQNLLNERKIIRAAQENGTVAINNRIPLQSLTAANIMVEGSIIGYESNVKSGGVGARYFGIGADTQYQLDQIAVNLRVVNVSTGEILSSVNTSKTILSYEVQAGVFRFIDYQRLLEGEIGYTSNEPVMLCLMSAIETGVIFLINDGIDRGLWDLQNKADRQNDILVKYRHMSVPPES

SEQ ID NO: 394 - protein, 262 aa, Citrobacter rodentium
CLTTPPKEAAKPTLMPRAQSYKDLTHLPVPTGKIFVSVYNIQDETGQFKPYPASNFSTAVPQSATAMLVTALKDSRWFIPLERQGLQNLLNERKIIRAAQENGTVAINNRIPLPSLTAANIMVEGSIIGYESNVKSGGAGARYFGIGADTQYQLDQIAVNLRVVNVSTGEILSSVNTSKTILSYEVQAGVFRFIDYQRLLEGEIGYTSNEPVMLCLMSAIETGVIFLINDGIDRGLWDLQNKADRQNDILVKYRQMSVPPES

SEQ ID NO: 395 - protein, 262 aa, Enterobacter asburiae
CLTAPPKEAAKPTLMPRAQSYRDLTHLPAPTGKIFVSVYNIQDETGQFKPYPASNFSTAVPQSATAMLVTALKDSHWFIPLERQGLQNLLNERKIIRAAQENGTVANNNRMPLQSLAAANVMIEGSIIGYESNVKSGGVGARYFGIGADTQYQLDQIAVNLRVVNVSTGEVLSSVNTSKTILSYEVQAGVFRFIDYQRLLEGEIGYTSNEPVMMCLMSAIETGVIFLINDGIDRGLWDLQNKADAQNPVLVKYRDMSVPPES

SEQ ID NO: 396 - DNA, 1830 bp, Bacillus subtilis phage phi29
atgaaacacatgccgcgtaaaatgtatagctgcgcgtttgaaaccacgaccaaagtggaagattgtcgcgtttgggcctatggctacatgaacatcgaagatcattctgaatacaaaatcggtaacagtctggatgaatttatggcatgggtgctgaaagttcaggcggatctgtacttccacaacctgaaatttgatggcgcattcattatcaactggctggaacgtaatggctttaaatggagcgcggatggtctgccgaacacgtataataccattatctctcgtatgggccagtggtatatgattgatatctgcctgggctacaaaggtaaacgcaaaattcataccgtgatctatgatagcctgaaaaaactgccgtttccggtgaagaaaattgcgaaagatttcaaactgacggttctgaaaggcgatattgattatcacaaagaacgtccggttggttacaaaatcaccccggaagaatacgcatacatcaaaaacgatatccagatcatcgcagaagcgctgctgattcagtttaaacagggcctggatcgcatgaccgcgggcagtgatagcctgaaaggtttcaaagatatcatcacgaccaaaaaattcaaaaaagtgttcccgacgctgagcctgggtctggataaagaagttcgttatgcctaccgcggcggttttacctggctgaacgatcgtttcaaagaaaaagaaattggcgagggtatggtgtttgatgttaatagtctgtatccggcacagatgtacagccgcctgctgccgtatggcgaaccgatcgtgttcgagggtaaatatgtttgggatgaagattacccgctgcatattcagcacatccgttgtgaatttgaactgaaagaaggctatattccgaccattcagatcaaacgtagtcgcttctataagggtaacgaatacctgaaaagctctggcggtgaaatcgcggatctgtggctgagtaacgtggatctggaactgatgaaagaacactacgatctgtacaacgttgaatacatcagcggcctgaaatttaaagccacgaccggtctgttcaaagatttcatcgataaatggacctacatcaaaacgacctctgaaggcgcgattaaacagctggccaaactgatgctgaacagcctgtatggcaaattcgcctctaatccggatgtgaccggtaaagttccgtacctgaaagaaaatggcgcactgggttttcgcctgggcgaagaagaaacgaaagatccggtgtataccccgatgggtgttttcattacggcctgggcacgttacacgaccatcaccgcggcccaggcatgctatgatcgcattatctactgtgataccgattctattcatctgacgggcaccgaaatcccggatgtgattaaagatatcgttgatccgaaaaaactgggttattgggcccacgaaagtacgtttaaacgtgcaaaatacctgcgccagaaaacctacatccaggatatctacatgaaagaagtggatggcaaactggttgaaggttctccggatgattacaccgatatcaaattcagtgtgaaatgcgccggcatgacggataaaatcaaaaaagaagtgaccttcgaaaacttcaaagttggtttcagccgcaaaatgaaaccgaaaccggtgcaggttccgggcggtgtggttctggtggatgatacgtttaccattaaatctggcggtagtgcgtggagccatccgcagttcgaaaaaggcggtggctctggtggcggttctggcggtagtgcctggagccacccgcagtttgaaaaataataa

SEQ ID NO: 397 - protein, 608 aa, Bacillus subtilis phage phi29
MKHMPRKMYSCAFETTTKVEDCRVWAYGYMNIEDHSEYKIGNSLDEFMAWVLKVQADLYFHNLKFDGAFIINWLERNGFKWSADGLPNTYNTIISRMGQWYMIDICLGYKGKRKIHTVIYDSLKKLPFPVKKIAKDFKLTVLKGDIDYHKERPVGYKITPEEYAYIKNDIQIIAEALLIQFKQGLDRMTAGSDSLKGFKDIITTKKFKKVFPTLSLGLDKEVRYAYRGGFTWLNDRFKEKEIGEGMVFDVNSLYPAQMYSRLLPYGEPIVFEGKYVWDEDYPLHIQHIRCEFELKEGYIPTIQIKRSRFYKGNEYLKSSGGEIADLWLSNVDLELMKEHYDLYNVEYISGLKFKATTGLFKDFIDKWTYIKTTSEGAIKQLAKLMLNSLYGKFASNPDVTGKVPYLKENGALGFRLGEEETKDPVYTPMGVFITAWARYTTITAAQACYDRIIYCDTDSIHLTGTEIPDVIKDIVDPKKLGYWAHESTFKRAKYLRQKTYIQDIYMKEVDGKLVEGSPDDYTDIKFSVKCAGMTDKIKKEVTFENFKVGFSRKMKPKPVQVPGGVVLVDDTFTIKSGGSAWSHPQFEKGGGSGGGSGGSAWSHPQFEK

SEQ ID NO: 398 - DNA, 1390 bp, Escherichia coli
atgatgaacgatggcaaacagcagagcaccttcctgtttcatgattatgaaaccttcggtacccatccggccctggatcgtccggcgcagtttgcggccattcgcaccgatagcgaattcaatgtgattggcgaaccggaagtgttttattgcaaaccggccgatgattatctgccgcagccgggtgcggtgctgattaccggtattaccccgcaggaagcgcgcgcgaaaggtgaaaacgaagcggcgtttgccgcgcgcattcatagcctgtttaccgtgccgaaaacctgcattctgggctataacaatgtgcgcttcgatgatgaagttacccgtaatatcttttatcgtaacttttatgatccgtatgcgtggagctggcagcatgataacagccgttgggatctgctggatgtgatgcgcgcgtgctatgcgctgcgcccggaaggcattaattggccggaaaacgatgatggcctgccgagctttcgtctggaacatctgaccaaagccaacggcattgaacatagcaatgcccatgatgcgatggccgatgtttatgcgaccattgcgatggcgaaactggttaaaacccgtcagccgcgcctgtttgattatctgtttacccaccgtaacaaacacaaactgatggcgctgattgatgttccgcagatgaaaccgctggtgcatgtgagcggcatgtttggcgcctggcgcggcaacaccagctgggtggccccgctggcctggcacccggaaaatcgtaacgccgtgattatggttgatctggccggtgatattagcccgctgctggaactggatagcgataccctgcgtgaacgcctgtataccgccaaaaccgatctgggcgataatgccgccgtgccggtgaaactggttcacattaacaaatgcccggtgctggcccaggcgaacaccctgcgcccggaagatgcggatcgtctgggtattaatcgccagcattgtctggataatctgaaaatcctgcgtgaaaacccgcaggtgcgtgaaaaagtggtggcgatcttcgcggaagcggaaccgttcaccccgagcgataacgtggatgcgcagctgtataacggcttctttagcgatgccgatcgcgcggcgatgaaaatcgttctggaaaccgaaccgcgcaatctgccggcgctggatattacctttgttgataaacgtattgaaaaactgctgtttaattatcgtgcgcgcaattttccgggtaccctggattatgccgaacagcagcgttggctggaacatcgtcgtcaggttttcaccccggaatttctgcagggttatgcggatgaactgcagatgctggttcagcagtatgccgatgataaagaaaaagtggcgctgc

SEQ ID NO: 399 - protein, 485 aa, Escherichia coli
MMNDGKQQSTFLFHDYETFGTHPALDRPAQFAAIRTDSEFNVIGEPEVFYCKPADDYLPQPGAVLITGITPQEARAKGENEAAFAARIHSLFTVPKTCILGYNNVRFDDEVTRNIFYRNFYDPYAWSWQHDNSRWDLLDVMRACYALRPEGINWPENDDGLPSFRLEHLTKANGIEHSNAHDAMADVYATIAMAKLVKTRQPRLFDYLFTHRNKHKLMALIDVPQMKPLVHVSGMFGAWRGNTSWVAPLAWHPENRNAVIMVDLAGDISPLLELDSDTLRERLYTAKTDLGDNAAVPVKLVHINKCPVLAQANTLRPEDADRLGINRQHCLDNLKILRENPQVREKVVAIFAEAEPFTPSDNVDAQLYNGFFSDADRAAMKIVLETEPRNLPALDITFVDKRIEKLLFNYRARNFPGTLDYAEQQRWLEHRRQVFTPEFLQGYADELQMLVQQYADDKEKVALLKALWQYAEEIVSGSGHHHHHH

SEQ ID NO: 400 - DNA, 804 bp, Escherichia coli
atgaaatttgtctcttttaatatcaacggcctgcgcgccagacctcaccagcttgaagccatcgtcgaaaagcaccaaccggatgtgattggcctgcaggagacaaaagttcatgacgatatgtttccgctcgaagaggtggcgaagctcggctacaacgtgttttatcacgggcagaaaggccattatggcgtggcgctgctgaccaaagagacgccgattgccgtgcgtcgcggctttcccggtgacgacgaagaggcgcagcggcggattattatggcggaaatcccctcactgctgggtaatgtcaccgtgatcaacggttacttcccgcagggtgaaagccgcgaccatccgataaaattcccggcaaaagcgcagttttatcagaatctgcaaaactacctggaaaccgaactcaaacgtgataatccggtactgattatgggcgatatgaatatcagccctacagatctggatatcggcattggcgaagaaaaccgtaagcgctggctgcgtaccggtaaatgctctttcctgccggaagagcgcgaatggatggacaggctgatgagctgggggttggtcgataccttccgccatgcgaatccgcaaacagcagatcgtttctcatggtttgattaccgctcaaaaggttttgacgataaccgtggtctgcgcatcgacctgctgctcgccagccaaccgctggcagaatgttgcgtagaaaccggcatcgactatgaaatccgcagcatggaaaaaccgtccgatcacgcccccgtctgggcgaccttccgccgc

SEQ ID NO: 401 - protein, 268 aa, Escherichia coli
MKFVSFNINGLRARPHQLEAIVEKHQPDVIGLQETKVHDDMFPLEEVAKLGYNVFYHGQKGHYGVALLTKETPIAVRRGFPGDDEEAQRRIIMAEIPSLLGNVTVINGYFPQGESRDHPIKFPAKAQFYQNLQNYLETELKRDNPVLIMGDMNISPTDLDIGIGEENRKRWLRTGKCSFLPEEREWMDRLMSWGLVDTFRHANPQTADRFSWFDYRSKGFDDNRGLRIDLLLASQPLAECCVETGIDYEIRSMEKPSDHAPVWATFRR

SEQ ID NO: 402 - DNA, 1275 bp, Thermus thermophilus
atgtttcgtcgtaaagaagatctggatccgccgctggcactgctgccgctgaaaggcctgcgcgaagccgccgcactgctggaagaagcgctgcgtcaaggtaaacgcattcgtgttcacggcgactatgatgcggatggcctgaccggcaccgcgatcctggttcgtggtctggccgccctgggtgcggatgttcatccgtttatcccgcaccgcctggaagaaggctatggtgtcctgatggaacgcgtcccggaacatctggaagcctcggacctgtttctgaccgttgactgcggcattaccaaccatgcggaactgcgcgaactgctggaaaatggcgtggaagtcattgttaccgatcatcatacgccgggcaaaacgccgccgccgggtctggtcgtgcatccggcgctgacgccggatctgaaagaaaaaccgaccggcgcaggcgtggcgtttctgctgctgtgggcactgcatgaacgcctgggcctgccgccgccgctggaatacgcggacctggcagccgttggcaccattgccgacgttgccccgctgtggggttggaatcgtgcactggtgaaagaaggtctggcacgcatcccggcttcatcttgggtgggcctgcgtctgctggctgaagccgtgggctataccggcaaagcggtcgaagtcgctttccgcatcgcgccgcgcatcaatgcggcttcccgcctgggcgaagcggaaaaagccctgcgcctgctgctgacggatgatgcggcagaagctcaggcgctggtcggcgaactgcaccgtctgaacgcccgtcgtcagaccctggaagaagcgatgctgcgcaaactgctgccgcaggccgacccggaagcgaaagccatcgttctgctggacccggaaggccatccgggtgttatgggtattgtggcctctcgcatcctggaagcgaccctgcgcccggtctttctggtggcccagggcaaaggcaccgtgcgttcgctggctccgatttccgccgtcgaagcactgcgcagcgcggaagatctgctgctgcgttatggtggtcataaagaagcggcgggtttcgcaatggatgaagcgctgtttccggcgttcaaagcacgcgttgaagcgtatgccgcacgtttcccggatccggttcgtgaagtggcactgctggatctgctgccggaaccgggcctgctgccgcaggtgttccgtgaactggcactgctggaaccgtatggtgaaggtaacccggaaccgctgttcctg

SEQ ID NO: 403 - protein, 425 aa, Thermus thermophilus
MFRRKEDLDPPLALLPLKGLREAAALLEEALRQGKRIRVHGDYDADGLTGTAILVRGLAALGADVHPFIPHRLEEGYGVLMERVPEHLEASDLFLTVDCGITNHAELRELLENGVEVIVTDHHTPGKTPPPGLVVHPALTPDLKEKPTGAGVAFLLLWALHERLGLPPPLEYADLAAVGTIADVAPLWGWNRALVKEGLARIPASSWVGLRLLAEAVGYTGKAVEVAFRIAPRINAASRLGEAEKALRLLLTDDAAEAQALVGELHRLNARRQTLEEAMLRKLLPQADPEAKAIVLLDPEGHPGVMGIVASRILEATLRPVFLVAQGKGTVRSLAPISAVEALRSAEDLLLRYGGHKEAAGFAMDEALFPAFKARVEAYAARFPDPVREVALLDLLPEPGLLPQVFRELALLEPYGEGNPEPLFL

SEQ ID NO: 404 - DNA, 738 bp, Bacteriophage lambda
tccggaagcggctctggtagtggttctggcatgacaccggacattatcctgcagcgtaccgggatcgatgtgagagctgtcgaacagggggatgatgcgtggcacaaattacggctcggcgtcatcaccgcttcagaagttcacaacgtgatagcaaaaccccgctccggaaagaagtggcctgacatgaaaatgtcctacttccacaccctgcttgctgaggtttgcaccggtgtggctccggaagttaacgctaaagcactggcctggggaaaacagtacgagaacgacgccagaaccctgtttgaattcacttccggcgtgaatgttactgaatccccgatcatctatcgcgacgaaagtatgcgtaccgcctgctctcccgatggtttatgcagtgacggcaacggccttgaactgaaatgcccgtttacctcccgggatttcatgaagttccggctcggtggtttcgaggccataaagtcagcttacatggcccaggtgcagtacagcatgtgggtgacgcgaaaaaatgcctggtactttgccaactatgacccgcgtatgaagcgtgaaggcctgcattatgtcgtgattgagcgggatgaaaagtacatggcgagttttgacgagatcgtgccggagttcatcgaaaaaatggacgaggcactggctgaaattggttttgtatttggggagcaatggcgatctggctctggttccggcagcggttccgga

SEQ ID NO: 405 - protein, 226 aa, Bacteriophage lambda
MTPDIILQRTGIDVRAVEQGDDAWHKLRLGVITASEVHNVIAKPRSGKKWPDMKMSYFHTLLAEVCTGVAPEVNAKALAWGKQYENDARTLFEFTSGVNVTESPIIYRDESMRTACSPDGLCSDGNGLELKCPFTSRDFMKFRLGGFEAIKSAYMAQVQYSMWVTRKNAWYFANYDPRMKREGLHYVVIERDEKYMASFDEIVPEFIEKMDEALAEIGFVFGEQWR

SEQ ID NO: 406 - protein, 760 aa, Methanococcoides burtonii
MMIRELDIPRDIIGFYEDSGIKELYPPQAEAIEMGLLEKKNLLAAIPTASGKTLLAELAMIKAIREGGKALYIVPLRALASEKFERFKELAPFGIKVGISTGDLDSRADWLGVNDIIVATSEKTDSLLRNGTSWMDEITTVVVDEIHLLDSKNRGPTLEVTITKLMRLNPDVQVVALSATVGNAREMADWLGAALVLSEWRPTDLHEGVLFGDAINFPGSQKKIDRLEKDDAVNLVLDTIKAEGQCLVFESSRRNCAGFAKTASSKVAKILDNDIMIKLAGIAEEVESTGETDTAIVLANCIRKGVAFHHAGLNSNHRKLVENGFRQNLIKVISSTPTLAAGLNLPARRVIIRSYRRFDSNFGMQPIPVLEYKQMAGRAGRPHLDPYGESVLLAKTYDEFAQLMENYVEADAEDIWSKLGTENALRTHVLSTIVNGFASTRQELFDFFGATFFAYQQDKWMLEEVINDCLEFLIDKAMVSETEDIEDASKLFLRGTRLGSLVSMLYIDPLSGSKIVDGFKDIGKSTGGNMGSLEDDKGDDITVTDMTLLHLVCSTPDMRQLYLRNTDYTIVNEYIVAHSDEFHEIPDKLKETDYEWFMGEVKTAMLLEEWVTEVSAEDITRHFNVGEGDIHALADTSEWLMHAAAKLAELLGVEYSSHAYSLEKRIRYGSGLDLMELVGIRGVGRVRARKLYNAGFVSVAKLKGADISVLSKLVGPKVAYNILSGIGVRVNDKHFNSAPISSNTLDTLLDKNQKTFNDFQ

SEQ ID NO: 407 - protein, 707 aa, Cenarchaeum symbiosum
MRISELDIPRPAIEFLEGEGYKKLYPPQAAAAKAGLTDGKSVLVSAPTASGKTLIAAIAMISHLSRNRGKAVYLSPLRALAAEKFAEFGKIGGIPLGRPVRVGVSTGDFEKAGRSLGNNDILVLTNERMDSLIRRRPDWMDEVGLVIADEIHLIGDRSRGPTLEMVLTKLRGLRSSPQVVALSATISNADEIAGWLDCTLVHSTWRPVPLSEGVYQDGEVAMGDGSRHEVAATGGGPAVDLAAESVAEGGQSLIFADTRARSASLAAKASAVIPEAKGADAAKLAAAAKKIISSGGETKLAKTLAELVEKGAAFHHAGLNQDCRSVVEEEFRSGRIRLLASTPTLAAGVNLPARRVVISSVMRYNSSSGMSEPISILEYKQLCGRAGRPQYDKSGEAIVVGGVNADEIFDRYIGGEPEPIRSAMVDDRALRIHVLSLVTTSPGIKEDDVTEFFLGTLGGQQSGESTVKFSVAVALRFLQEEGMLGRRGGRLAATKMGRLVSRLYMDPMTAVTLRDAVGEASPGRMHTLGFLHLVSECSEFMPRFALRQKDHEVAEMMLEAGRGELLRPVYSYECGRGLLALHRWIGESPEAKLAEDLKFESGDVHRMVESSGWLLRCIWEISKHQERPDLLGELDVLRSRVAYGIKAELVPLVSIKGIGRVRSRRLFRGGIKGPGDLAAVPVERLSRVEGIGATLANNIKSQLRKGG

SEQ ID NO: 408 - protein, 720 aa, Thermococcus gammatolerans
MKVDELPVDERLKAVLKERGIEELYPPQAEALKSGALEGRNLVLAIPTASGKTLVSEIVMVNKLIQEGGKAVYLVPLKALAEEKYREFKEWEKLGLKVAATTGDYDSTDDWLGRYDIIVATAEKFDSLLRHGARWINDVKLVVADEVHLIGSYDRGATLEMILTHMLGRAQILALSATVGNAEELAEWLDASLVVSDWRPVQLRRGVFHLGTLIWEDGKVESYPENWYSLVVDAVKRGKGALVFVNTRRSAEKEALALSKLVSSHLTKPEKRALESLASQLEDNPTSEKLKRALRGGVAFHHAGLSRVERTLIEDAFREGLIKVITATPTLSAGVNLPSFRVIIRDTKRYAGFGWTDIPVLEIQQMMGRAGRPRYDKYGEAIIVARTDEPGKLMERYIRGKPEKLFSMLANEQAFRSQVLALITNFGIRSFPELVRFLERTFYAHQRKDLSSLEYKAKEVVYFLIENEFIDLDLEDRFIPLPFGKRTSQLYIDPLTAKKFKDAFPAIERNPNPFGIFQLIASTPDMATLTARRREMEDYLDLAYELEDKLYASIPYYEDSRFQGFLGQVKTAKVLLDWINEVPEARIYETYSIDPGDLYRLLELADWLMYSLIELYKLFEPKEEILNYLRDLHLRLRHGVREELLELVRLPNIGRKRARALYNAGFRSVEAIANAKPAELLAVEGIGAKILDGIYRHLGIEKRVTEEKPKRKGTLEDFLR

SEQ ID NO: 409 - protein, 799 aa, Methanospirillum hungatei
MEIASLPLPDSFIRACHAKGIRSLYPPQAECIEKGLLEGKNLLISIPTASGKTLLAEMAMWSRIAAGGKCLYIVPLRALASEKYDEFSKKGVIRVGIATGDLDRTDAYLGENDIIVATSEKTDSLLRNRTPWLSQITCIVLDEVHLIGSENRGATLEMVITKLRYTNPVMQIIGLSATIGNPAQLAEWLDATLITSTWRPVDLRQGVYYNGKIRFSDSERPIQGKTKHDDLNLCLDTIEEGGQCLVFVSSRRNAEGFAKKAAGALKAGSPDSKALAQELRRLRDRDEGNVLADCVERGAAFHHAGLIRQERTIIEEGFRNGYIEVIAATPTLAAGLNLPARRVIIRDYNRFASGLGMVPIPVGEYHQMAGRAGRPHLDPYGEAVLLAKDAPSVERLFETFIDAEAERVDSQCVDDASLCAHILSLIATGFAHDQEALSSFMERTFYFFQHPKTRSLPRLVADAIRFLTTAGMVEERENTLSATRLGSLVSRLYLNPCTARLILDSLKSCKTPTLIGLLHVICVSPDMQRLYLKAADTQLLRTFLFKHKDDLILPLPFEQEEEELWLSGLKTALVLTDWADEFSEGMIEERYGIGAGDLYNIVDSGKWLLHGTERLVSVEMPEMSQVVKTLSVRVHHGVKSELLPLVALRNIGRVRARTLYNAGYPDPEAVARAGLSTIARIIGEGIARQVIDEITGVKRSGIHSSDDDYQQKTPELLTDIPGIGKKMAEKLQNAGIITVSDLLTADEVLLSDVLGAARARKVLAFLSNSEKENSSSDKTEEIPDTQKIRGQSSWEDFGC

SEQ ID NO: 410 - protein, 1756 aa, Escherichia coli
MMSIAQVRSAGSAGNYYTDKDNYYVLGSMGERWAGKGAEQLGLQGSVDKDVFTRLLEGRLPDGADLSRMQDGSNKHRPGYDLTFSAPKSVSMMAMLGGDKRLIDAHNQAVDFAVRQVEALASTRVMTDGQSETVLTGNLVMALFNHDTSRDQEPQLHTHAVVANVTQHNGEWKTLSSDKVGKTGFIENVYANQIAFGRLYREKLKEQVEALGYETEVVGKHGMWEMPGVPVEAFSGRSQAIREAVGEDASLKSRDVAALDTRKSKQHVDPEIRMAEWMQTLKETGFDIRAYRDAADQRTEIRTQAPGPASQDGPDVQQAVTQAIAGLSERKVQFTYTDVLARTVGILPPENGVIERARAGIDEAISREQLIPLDREKGLFTSGIHVLDELSVRALSRDIMKQNRVTVHPEKSVPRTAGYSDAVSVLAQDRPSLAIVSGQGGAAGQRERVAELVMMAREQGREVQIIAADRRSQMNLKQDERLSGELITGRRQLLEGMAFTPGSTVIVDQGEKLSLKETLTLLDGAARHNVQVLITDSGQRTGTGSALMAMKDAGVNTYRWQGGEQRPATIISEPDRNVRYARLAGDFAASVKAGEESVAQVSGVREQAILTQAIRSELKTQGVLGHPEVTMTALSPVWLDSRSRYLRDMYRPGMVMEQWNPETRSHDRYVIDRVTAQSHSLTLRDAQGETQVVRISSLDSSWSLFRPEKMPVADGERLRVTGKIPGLRVSGGDRLQVASVSEDAMTVVVPGRAEPASLPVSDSPFTALKLENGWVETPGHSVSDSATVFASVTQMAMDNATLNGLARSGRDVRLYSSLDETRTAEKLARHPSFTVVSEQIKARAGETLLETAISLQKAGLHTPAQQAIHLALPVLESKNLAFSMVDLLTEAKSFAAEGTGFTELGGEINAQIKRGDLLYVDVAKGYGTGLLVSRASYEAEKSILRHILEGKEAVTPLMERVPGELMETLTSGQRAATRMILETSDRFTVVQGYAGVGKTTQFRAVMSAVNMLPASERPRVVGLGPTHRAVGEMRSAGVDAQTLASFLHDTQLQQRSGETPDFSNTLFLLDESSMVGNTEMARAYALIAAGGGRAVASGDTDQLQAIAPGQSFRLQQTRSAADVVIMKEIVRQTPELREAVYSLINRDVERALSGLESVKPSQVPRLEGAWAPEHSVTEFSHSQEAKLAEAQQKAMLKGEAFPDIPMTLYEAIVRDYTGRTPEAREQTLIVTHLNEDRRVLNSMIHDAREKAGELGKEQVMVPVLNTANIRDGELRRLSTWEKNPDALALVDNVYHRIAGISKDDGLITLQDAEGNTRLISPREAVAEGVTLYTPDKIRVGTGDRMRFTKSDRERGYVANSVWTVTAVSGDSVTLSDGQQTRVIRPGQERAEQHIDLAYAITAHGAQGASETFAIALEGTEGNRKLMAGFESAYVALSRMKQHVQVYTDNRQGWTDAINNAVQKGTAHDVLEPKPDREVMNAQRLFSTARELRDVAAGRAVLRQAGLAGGDSPARFIAPGRKYPQPYVALPAFDRNGKSAGIWLNPLTTDDGNGLRGFSGEGRVKGSGDAQFVALQGSRNGESLLADNMQDGVRIARDNPDSGVVVRIAGEGRPWNPGAITGGRVWGDIPDNSVQPGAGNGEPVTAEVLAQRQAEEAIRRETERRADEIVRKMAENKPDLPDGKTELAVRDIAGQERDRSAISERETALPESVLRESQREREAVREVARENLLQERLQQMERDMVRDLQKEKTLGGD

SEQ ID NO: 411 - protein, 726 aa, Methanococcoides burtonii
MSDKPAFMKYFTQSSCYPNQQEAMDRIHSALMQQQLVLFEGACGTGKTLSALVPALHVGKMLGKTVIIATNVHQQMVQFINEARDIKKVQDVKVAVIKGKTAMCPQEADYEECSVKRENTFELMETEREIYLKRQELNSARDSYKKSHDPAFVTLRDELSKEIDAVEEKARGLRDRACNDLYEVLRSDSEKFREWLYKEVRSPEEINDHAIKDGMCGYELVKRELKHADLLICNYHHVLNPDIFSTVLGWIEKEPQETIVIFDEAHNLESAARSHSSLSLTEHSIEKAITELEANLDLLADDNIHNLFNIFLEVISDTYNSRFKFGERERVRKNWYDIRISDPYERNDIVRGKFLRQAKGDFGEKDDIQILLSEASELGAKLDETYRDQYKKGLSSVMKRSHIRYVADFMSAYIELSHNLNYYPILNVRRDMNDEIYGRVELFTCIPKNVTEPLFNSLFSVILMSATLHPFEMVKKTLGITRDTCEMSYGTSFPEEKRLSIAVSIPPLFAKNRDDRHVTELLEQVLLDSIENSKGNVILFFQSAFEAKRYYSKIEPLVNVPVFLDEVGISSQDVREEFFSIGEENGKAVLLSYLWGTLSEGIDYRDGRGRTVIIIGVGYPALNDRMNAVESAYDHVFGYGAGWEFAIQVPTIRKIRQAMGRVVRSPTDYGARILLDGRFLTDSKKRFGKFSVFEVFPPAERSEFVDVDPEKVKYSLMNFFMDNDEQ

SEQ ID NO: 412 - protein, 439 aa, Bacteriophage T4
MTFDDLTEGQKNAFNIVMKAIKEKKHHVTINGPAGTGKTTLTKFIIEALISTGETGIILAAPTHAAKKILSKLSGKEASTIHSILKINPVTYEENVLFEQKEVPDLAKCRVLICDEVSMYDRKLFKILLSTIPPWCTIIGIGDNKQIRPVDPGENTAYISPFFTHKDFYQCELTEVKRSNAPIIDVATDVRNGKWIYDKVVDGHGVRGFTGDTALRDFMVNYFSIVKSLDDLFENRVMAFTNKSVDKLNSIIRKKIFETDKDFIVGEIIVMQEPLFKTYKIDGKPVSEIIFNNGQLVRIIEAEYTSTFVKARGVPGEYLIRHWDLTVETYGDDEYYREKIKIISSDEELYKFNLFLGKTAETYKNWNKGGKAPWSDFWDAKSQFSKVKALPASTFHKAQGMSVDRAFIYTPCIHYADVELAQQLLYVGVTRGRYDVFYV

SEQ ID NO: 413 - protein, 970 aa, Citromicrobium bathyomarinum
MLSVANVRSPSAAASYFASDNYYASADADRSGQWIGDGAKRLGLEGKVEARAFDALLRGELPDGSSVGNPGQAHRPGTDLTFSVPKSWSLLALVGKDERIIAAYREAVVEALHWAEKNAAETRVVEKGMVVTQATGNLAIGLFQHDTNRNQEPNLHFHAVIANVTQGKDGKWRTLKNDRLWQLNTTLNSIAMARFRVAVEKLGYEPGPVLKHGNFEARGISREQVMAFSTRRKEVLEARRGPGLDAGRIAALDTRASKEGIEDRATLSKQWSEAAQSIGLDLKPLVDRARTKALGQGMEATRIGSLVERGRAWLSRFAAHVRGDPADPLVPPSVLKQDRQTIAAAQAVASAVRHLSQREAAFERTALYKAALDFGLPTTIADVEKRTRALVRSGDLIAGKGEHKGWLASRDAVVTEQRILSEVAAGKGDSSPAITPQKAAASVQAAALTGQGFRLNEGQLAAARLILISKDRTIAVQGIAGAGKSSVLKPVAEVLRDEGHPVIGLAIQNTLVQMLERDTGIGSQTLARFLGGWNKLLDDPGNVALRAEAQASLKDHVLVLDEASMVSNEDKEKLVRLANLAGVHRLVLIGDRKQLGAVDAGKPFALLQRAGIARAEMATNLRARDPVVREAQAAAQAGDVRKALRHLKSHTVEARGDGAQVAAETWLALDKETRARTSIYASGRAIRSAVNAAVQQGLLASREIGPAKMKLEVLDRVNTTREELRHLPAYRAGRVLEVSRKQQALGLFIGEYRVIGQDRKGKLVEVEDKRGKRFRFDPARIRAGKGDDNLTLLEPRKLEIHEGDRIRWTRNDHRRGLFNADQARVVEIANGKVTFETSKGDLVELKKDDPMLKRIDLAYALNVHMAQGLTSDRGIAVMDSRERNLSNQKTFLVTVTRLRDHLTLVVDSADKLGAAVARNKGEKASAIEVTGSVKPTATKGSGVDQPKSVEANKAEKELTRSKSKTLDFGI

SEQ ID NO: 414 - protein, 262 aa, Yokenella regensburgei
CLTAPPKEAAKPTLMPRAQSYRDLTHLPLPSGKVFVSVYNIQDETGQFKPYPASNFSTAVPQSATAMLVTALKDSRWFVPLERQGLQNLLNERKIIRAAQENGTVADNNRIPLQSLTAANVMIEGSIIGYESNVKSGGVGARYFGIGADTQYQLDQIAVNLRVVNVSTGEVLSSVNTSKTILSYEVQAGVFRFVDYQRLLEGEIGYTSNEPVMLCLMSAIETGVIYLINDGIERGLWDLQQKADVDNPILARYRNMSAPPES

SEQ ID NO: 415 - protein, 262 aa, Cronobacter pulveris
CLTAPPKEAAKPTLMPRAQSYRDLTNLPDPKGKLFVSVYNIQDETGQFKPYPASNFSTAVPQSATSMLVTALKDSRWFIPLERQGLQNLLNERKIIRAAQENGTVAENNRMPLQSLVAANVMIEGSIIGYESNVKSGGVGARYFGIGGDTQYQLDQIAVNLRVVNVSTGEVLSSVNTSKTILSYEVQAGVFRFIDYQRLLEGEIGYTANEPVMLCLMSAIETGVIHLINDGINRGLWELKNKGDAKNTILAKYRSMAVPPES

SEQ ID NO: 416 - protein, 262 aa, Rahnella aquatilis
CLTAAPKEAARPTLLPRAPSYTDLTHLPSPQGRIFVSVYNIQDETGQFKPYPACNFSTAVPQSATAMLVSALKDSKWFIPLERQGLQNLLNERKIIRAAQENGSVAINNQRPLSSLVAANILIEGSIIGYESNVKSGGVGARYFGIGASTQYQLDQIAVNLRAVDVNTGEVLSSVNTSKTILSYEVQAGVFRFIDYQRLLEGELGYTTNEPVMLCLMSAIESGVIYLVNDGIERNLWQLQNPSEINSPILQRYKNNIVPAES

SEQ ID NO: 417 - protein, 259 aa, Kluyvera ascorbata
CITSPPKQAAKPTLLPRSQSYQDLTHLPEPQGRLFVSVYNISDETGQFKPYPASNFSTSVPQSATAMLVSALKDSNWFIPLERQGLQNLLNERKIIRAAQENGTVAVNNRTQLPSLVAANILIEGSIIGYESNVKSGGAGARYFGIGASTQYQLDQIAVNLRVVNVSTGEVLSSVNTSKTILSYEFQAGVFRYIDYQRLLEGEVGYTVNEPVMLCLMSAIETGVIYLVNDGISRNLWQLKNASDINSPVLEKYKSIIVP

SEQ ID NO: 418 - protein, 259 aa, Hafnia alvei
CLTAPPKQAAKPTLMPRAQSYQDLTHLPEPAGKLFVSVYNIQDETGQFKPYPASNFSTAVPQSATAMLVSALKDSGWFIPLERQGLQNLLNERKIIRAAQENGTAAVNNQHQLSSLVAANVLVEGSIIGYESNVKSGGAGARFFGIGASTQYQLDQIAVNLRVVDVNTGQVLSSVNTSKTILSYEVQAGVFRYIDYQRLLEGEIGYTTNEPVMLCVMSAIETGVIYLVNDGINRNLWTLKNPQDAKSSVLERYKSTIVP

SEQ ID NO: 419 - protein, 255 aa, Enterobacteriaceae bacterium strain FGI 57
CITTPPQEAAKPTLLPRDATYKDLVSLPQPRGKIYVAVYNIQDETGQFQPYPASNFSTSVPQSATAMLVSSLKDSRWFVPLERQGLNNLLNERKIIRAAQQNGTVGDNNASPLPSLYSANVIVEGSIIGYASNVKTGGFGARYFGIGGSTQYQLDQVAVNLRIVNVHTGEVLSSVNTSKTILSYEIQAGVFRFIDYQRLLEGEAGFTTNEPVMTCLMSAIEEGVIHLINDGINKKLWALSNAADINSEVLTRYRK

SEQ ID NO: 420 - protein, 258 aa, Plesiomonas shigelloides
ITEVPKEAAKPTLMPRASTYKDLVALPKPNGKIIVSVYSVQDETGQFKPLPASNFSTAVPQSGNAMLTSALKDSGWFVPLEREGLQNLLNERKIIRAAQENGTVAANNQQPLPSLLSANVVIEGAIIGYDSDIKTGGAGARYFGIGADGKYRVDQVAVNLRAVDVRTGEVLLSVNTSKTILSSELSAGVFRFIEYQRLLELEAGYTTNEPVMMCMMSALEAGVAHLIVEGIRQNLWSLQNPSDINNPIIQRYMKEDVP

SEQ ID NO: 421 - protein, 248 aa, Vibrio fischeri
PETSESPTLMQRGANYIDLISLPKPQGKIFVSVYDFRDQTGQYKPQPNSNFSTAVPQGGTALLTMALLDSEWFYPLERQGLQNLLTERKIIRAAQKKQESISNHGSTLPSLLSANVMIEGGIVAYDSNIKTGGAGARYLGIGGSGQYRADQVTVNIRAVDVRSGKILTSVTTSKTILSYEVSAGAFRFVDYKELLEVELGYTNNEPVNIALMSAIDSAVIHLIVKGVQQGLWRPANLDTRNNPIFKKY

SEQ ID NO: 422 - protein, 248 aa, Aliivibrio logei
PDASESPTLMQRGATYLDLISLPKPQGKIYVSVYDFRDQTGQYKPQPNSNFSTAVPQGGTALLTMALLDSEWFYPLERQGLQNLLTERKIIRAAQKKQESISNHGSTLPSLLSANVMIEGGIVAYDSNIKTGGAGARYLGIGGSGQYRADQVTVNIRAVDVRSGKILTSVTTSKTILSYELSAGAFRFVDYKELLEVELGYTNNEPVNIALMSAIDSAVIHLIVKGIEEGLWRPENQNGKENPIFRKY

SEQ ID NO: 423 - protein, 254 aa, Photobacterium sp. AK15
PETSKEPTLMARGTAYQDLVSLPLPKGKVYVSVYDFRDQTGQYKPQPNSNFSTAVPQGGAALLTTALLDSRWFMPLEREGLQNLLTERKIIRAAQKKDEIPTNHGVHLPSLASANIMVEGGIVAYDTNIQTGGAGARYLGVGASGQYRTDQVTVNIRAVDVRTGRILLSVTTSKTILSKELQTGVFKFVDYKDLLEAELGYTTNEPVNLAVMSAIDAAVVHVIVDGIKTGLWEPLRGEDLQHPIIQEYMNRSKP

SEQ ID NO: 424 - protein, 261 aa, Aeromonas veronii
CATHIGSPVADEKATLMPRSVSYKELISLPKPKGKIVAAVYDFRDQTGQYLPAPASNFSTAVTQGGVAMLSTALWDSQWFVPLEREGLQNLLTERKIVRAAQNKPNVPGNNANQLPSLVAANILIEGGIVAYDSNVRTGGAGAKYFGIGASGEYRVDQVTVNLRAVDIRSGRILNSVTTSKTVMSQQVQAGVFRFVEYKRLLEAEAGFSTNEPVQMCVMSAIESGVIRLIANGVRDNLWQLADQRDIDNPILQEYLQDNAP

SEQ ID NO: 425 - protein, 239 aa, Shewanella sp. ECSMB14101
ASSSLMPKGESYYDLINLPAPQGVMLAAVYDFRDQTGQYKPIPSSNFSTAVPQSGTAFLAQALNDSSWFIPVEREGLQNLLTERKIVRAGLKGDANKLPQLNSAQILMEGGIVAYDTNVRTGGAGARYLGIGAATQFRVDTVTVNLRAVDIRTGRLLSSVTTTKSILSKEITAGVFKFIDAQELLESELGYTSNEPVSLCVASAIESAVVHMIADGIWKGAWNLADQASGLRSPVLQKY

SEQ ID NO: 426 - protein, 233 aa, Pseudomonas putida
QDSETPTLTPRASTYYDLINMPRPKGRLMAVVYGFRDQTGQYKPTPASSFSTSVTQGAASMLMDALSASGWFVVLEREGLQNLLTERKIIRASQKKPDVAENIMGELPPLQAANLMLEGGIIAYDTNVRSGGEGARYLGIDISREYRVDQVTVNLRAVDVRTGQVLANVMTSKTIYSVGRSAGVFKFIEFKKLLEAEVGYTTNEPAQLCVLSAIESAVGHLLAQGIEQRLWQV

SEQ ID NO: 427 - protein, 234 aa, Shewanella violacea DSS12
MPKSDTYYDLIGLPHPQGSMLAAVYDFRDQTGQYKAIPSSNFSTAVPQSGTAFLAQALNDSSWFVPVEREGLQNLLTERKIVRAGLKGEANQLPQLSSAQILMEGGIVAYDTNIKTGGAGARYLGIGVNSKFRVDTVTVNLRAVDIRTGRLLSSVTTTKSILSKEVSAGVFKFIDAQDLLESELGYTSNEPVSLCVAQAIESAVVHMIADGIWKRAWNLADTASGLNNPVLQKY

SEQ ID NO: 428 - protein, 245 aa, Marinobacterium jannaschii
LTRRMSTYQDLIDMPAPRGKIVTAVYSFRDQSGQYKPAPSSSFSTAVTQGAAAMLVNVLNDSGWFIPLEREGLQNILTERKIIRAALKKDNVPVNNSAGLPSLLAANIMLEGGIVGYDSNIHTGGAGARYFGIGASEKYRVDEVTVNLRAIDIRTGRILHSVLTSKKILSREIRSDVYRFIEFKHLLEMEAGITTNDPAQLCVLSAIESAVAHLIVDGVIKKSWSLADPNELNSPVIQAYQQQRI

SEQ ID NO: 429 - protein, 234 aa, Chryseobacterium oranimense G311
PSDPERSTMGELTPSTAELRNLPLPNEKIVIGVYKFRDQTGQYKPSENGNNWSTAVPQGTTTILIKALEDSRWFIPIERENIANLLNERQIIRSTRQEYMKDADKNSQSLPPLLYAGILLEGGVISYDSNTMTGGFGARYFGIGASTQYRQDRITIYLRAVSTLNGEILKTVYTSKTILSTSVNGSFFRYIDTERLLEAEVGLTQNEPVQLAVTEAIEKAVRSLIIEGTRDKIW

SEQ ID NO: 430 - DNA, 12 bp, artificial sequence
  polynucleotide sequence used in Example 18
tttttttttttt

SEQ ID NO: 431 - DNA, 27 bp, artificial sequence
  polynucleotide sequence used in Example 18
ggttgtttctgttggtgctgatattgc

SEQ ID NO: 432 - DNA, 3635 bp, artificial sequence
  polynucleotide sequence used in Example 18
gccatcagattgtgtttgttagtcgctgccatcagattgtgtttgttagtcgctttttttttttggaattttttttttggaattttttttttgcgctaacaacctcctgccgttttgcccgtgcatatcggtcacgaacaaatctgattactaaacacagtagcctggatttgttctatcagtaatcgaccttattcctaattaaatagagcaaatccccttattgggggtaagacatgaagatgccagaaaaacatgacctgttggccgccattctcgcggcaaaggaacaaggcatcggggcaatccttgcgtttgcaatggcgtaccttcgcggcagatataatggcggtgcgtttacaaaaacagtaatcgacgcaacgatgtgcgccattatcgcctagttcattcgtgaccttctcgacttcgccggactaagtagcaatctcgcttatataacgagcgtgtttatcggctacatcggtactgactcgattggttcgcttatcaaacgcttcgctgctaaaaaagccggagtagaagatggtagaaatcaataatcaacgtaaggcgttcctcgatatgctggcgtggtcggagggaactgataacggacgtcagaaaaccagaaatcatggttatgacgtcattgtaggcggagagctatttactgattactccgatcaccctcgcaaacttgtcacgctaaacccaaaactcaaatcaacaggcgccggacgctaccagcttctttcccgttggtgggatgcctaccgcaagcagcttggcctgaaagacttctctccgaaaagtcaggacgctgtggcattgcagcagattaaggagcgtggcgctttacctatgattgatcgtggtgatatccgtcaggcaatcgaccgttgcagcaatatctgggcttcactgccgggcgctggttatggtcagttcgagcataaggctgacagcctgattgcaaaattcaaagaagcgggcggaacggtcagagagattgatgtatgagcagagtcaccgcgattatctccgctctggttatctgcatcatcgtctgcctgtcatgggctgttaatcattaccgtgataacgccattacctacaaagcccagcgcgacaaaaatgccagagaactgaagctggcgaacgcggcaattactgacatgcagatgcgtcagcgtgatgttgctgcgctcgatgcaaaatacacgaaggagttagctgatgctaaagctgaaaatgatgctctgcgtgatgatgttgccgctggtcgtcgtcggttgcacatcaaagcagtctgtcagtcagtgcgtgaagccaccaccgcctccggcgtggataatgcagcctccccccgactggcagacaccgctgaacgggattatttcaccctcagagagaggctgatcactatgcaaaaacaactggaaggaacccagaagtatattaatgagcagtgcagatagagttgcccatatcgatgggcaactcatgcaattattgtgagcaatacacacgcgcttccagcggagtataaatgcctaaagtaataaaaccgagcaatccatttacgaatgtttgctgggtttctgttttaacaacattttctgcgccgccacaaattttggctgcatcgacagttttcttctgcccaattccagaaacgaagaaatgatgggtgatggtttcctttggtgctactgctgccggtttgttttgaacagtaaacgtctgttgagcacatcctgtaataagcagggccagcgcagtagcgagtagcatttttttcatggtgttattcccgatgctttttgaagttcgcagaatcgtatgtgtagaaaattaaacaaaccctaaacaatgagttgaaatttcatattgttaatatttattaatgtatgtcaggtgcgatgaatcgtcattgtattcccggattaactatgtccacagccctgacggggaacttctctgcgggagtgtccgggaataattaaaacgatgcacacagggtttagcgcgtacacgtattgcattatgccaacgccccggtgctgacacggaagaaaccggacgttatgatttagcgtggaaagatttgtgtagtgttctgaatgctctcagtaaatagtaatgaattatcaaaggtatagtaatatcttttatgttcatggatatttgtaacccatcggaaaactcctgctttagcaagattttccctgtattgctgaaatgtgatttctcttgatttcaacctatcataggacgtttctataagatgcgtgtttcttgagaatttaacatttacaacctttttaagtccttttattaacacggtgttatcgttttctaacacgatgtgaatattatctgtggctagatagtaaatataatgtgagacgttgtgacgttttagttcagaataaaacaattcacagtctaaatcttttcgcacttgatcgaatatttctttaaaaatggcaacctgagccattggtaaaaccttccatgtgatacgagggcgcgtagtttgcattatcgtttttatcgtttcaatctggtctgacctccttgtgttttgttgatgatttatgtcaaatattaggaatgttttcacttaatagtattggttgcgtaacaaagtgcggtcctgctggcattctggagggaaatacaaccgacagatgtatgtaaggccaacgtgctcaaatcttcatacagaaagatttgaagtaatattttaaccgctagatgaagagcaagcgcatggagcgacaaaatgaataaagaacaatctgctgatgatccctccgtggatctgattcgtgtaaaaaatatgcttaatagcaccatttctatgagttaccctgatgttgtaattgcatgtatagaacataaggtgtctctggaagcattcagagcaattgaggcagcgttggtgaagcacgataataatatgaaggattattccctggtggttgactgatcaccataactgctaatcattcaaactatttagtctgtgacagagccaacacgcagtctgtcactgtcaggaaagtggtaaaactgcaactcaattactgcaatgccctcgtaattaagtgaatttacaatatcgtcctgttcggagggaagaacgcgggatgttcattcttcatcacttttaattgatgtatatgctctcttttctgacgttagtctccgacggcaggcttcaatgacccaggctgagaaattcccggaccctttttgctcaagagcgatgttaatttgttcaatcatttggttaggaaagcggatgttgcgggttgttgttctgcgggttctgttcttcgttgacatgaggttgccccgtattcagtgtcgctgatttgtattgtctgaagttgtttttacgttaagttgatgcagatcaattaatacgatacctgcgtcataattgattatttgacgtggtttgatggcctccacgcacgttgtgatatgtagatgataatcattatcactttacgggtcctttccggtgaaaaaaaaggtaccaaaaaaaacatcgtcgtgagtagtgaaccgtaagccgttctgtttatgtttcttggacactgattgacacggtttagtagaac

SEQ ID NO: 433 - DNA, 3636 bp, artificial sequence
  polynucleotide sequence used in Example 18
ttttttttttttttttttttttttttttcaagaaacataaacagaacgtgcttacggttcactactcacgacgatgttttttttggtaccttttttttcaccggaaaggacccgtaaagtgataatgattatcatctacatatcacaacgtgcgtggaggccatcaaaccacgtcaaataatcaattatgacgcaggtatcgtattaattgatctgcatcaacttaacgtaaaaacaacttcagacaatacaaatcagcgacactgaatacggggcaacctcatgtcaacgaagaacagaacccgcagaacaacaacccgcaacatccgctttcctaaccaaatgattgaacaaattaacatcgctcttgagcaaaaagggtccgggaatttctcagcctgggtcattgaagcctgccgtcggagactaacgtcagaaaagagagcatatacatcaattaaaagtgatgaagaatgaacatcccgcgttcttccctccgaacaggacgatattgtaaattcacttaattacgagggcattgcagtaattgagttgcagttttaccactttcctgacagtgacagactgcgtgttggctctgtcacagactaaatagtttgaatgattagcagttatggtgatcagtcaaccaccagggaataatccttcatattattatcgtgcttcaccaacgctgcctcaattgctctgaatgcttccagagacaccttatgttctatacatgcaattacaacatcagggtaactcatagaaatggtgctattaagcatattttttacacgaatcagatccacggagggatcatcagcagattgttctttattcattttgtcgctccatgcgcttgctcttcatctagcggttaaaatattacttcaaatctttctgtatgaagatttgagcacgttggccttacatacatctgtcggttgtatttccctccagaatgccagcaggaccgcactttgttacgcaaccaatactattaagtgaaaacattcctaatatttgacataaatcatcaacaaaacacaaggaggtcagaccagattgaaacgataaaaacgataatgcaaactacgcgccctcgtatcacatggaaggttttaccaatggctcaggttgccatttttaaagaaatattcgatcaagtgcgaaaagatttagactgtgaattgttttattctgaactaaaacgtcacaacgtctcacattatatttactatctagccacagataatattcacatcgtgttagaaaacgataacaccgtgttaataaaaggacttaaaaaggttgtaaatgttaaattctcaagaaacacgcatcttatagaaacgtcctatgataggttgaaatcaagagaaatcacatttcagcaatacagggaaaatcttgctaaagcaggagttttccgatgggttacaaatatccatgaacataaaagatattactatacctttgataattcattactatttactgagagcattcagaacactacacaaatctttccacgctaaatcataacgtccggtttcttccgtgtcagcaccggggcgttggcataatgcaatacgtgtacgcgctaaaccctgtgtgcatcgttttaattattcccggacactcccgcagagaagttccccgtcagggctgtggacatagttaatccgggaatacaatgacgattcatcgcacctgacatacattaataaatattaacaatatgaaatttcaactcattgtttagggtttgtttaattttctacacatacgattctgcgaacttcaaaaagcatcgggaataacaccatgaaaaaaatgctactcgctactgcgctggccctgcttattacaggatgtgctcaacagacgtttactgttcaaaacaaaccggcagcagtagcaccaaaggaaaccatcacccatcatttcttcgtttctggaattgggcagaagaaaactgtcgatgcagccaaaatttgtggcggcgcagaaaatgttgttaaaacagaaacccagcaaacattcgtaaatggattgctcggttttattactttaggcatttatactccgctggaagcgcgtgtgtattgctcacaataattgcatgagttgcccatcgatatgggcaactctatctgcactgctcattaatatacttctgggttccttccagttgtttttgcatagtgatcagcctctctctgagggtgaaataatcccgttcagcggtgtctgccagtcggggggaggctgcattatccacgccggaggcggtggtggcttcacgcactgactgacagactgctttgatgtgcaaccgacgacgaccagcggcaacatcatcacgcagagcatcattttcagctttagcatcagctaactccttcgtgtattttgcatcgagcgcagcaacatcacgctgacgcatctgcatgtcagtaattgccgcgttcgccagcttcagttctctggcatttttgtcgcgctgggctttgtaggtaatggcgttatcacggtaatgattaacagcccatgacaggcagacgatgatgcagataaccagagcggagataatcgcggtgactctgctcatacatcaatctctctgaccgttccgcccgcttctttgaattttgcaatcaggctgtcagccttatgctcgaactgaccataaccagcgcccggcagtgaagcccagatattgctgcaacggtcgattgcctgacggatatcaccacgatcaatcataggtaaagcgccacgctccttaatctgctgcaatgccacagcgtcctgacttttcggagagaagtctttcaggccaagctgcttgcggtaggcatcccaccaacgggaaagaagctggtagcgtccggcgcctgttgatttgagttttgggtttagcgtgacaagtttgcgagggtgatcggagtaatcagtaaatagctctccgcctacaatgacgtcataaccatgatttctggttttctgacgtccgttatcagttccctccgaccacgccagcatatcgaggaacgccttacgttgattattgatttctaccatcttctactccggcttttttagcagcgaagcgtttgataagcgaaccaatcgagtcagtaccgatgtagccgataaacacgctcgttatataagcgagattgctacttagtccggcgaagtcgagaaggtcacgaatgaactaggcgataatggcgcacatcgttgcgtcgattactgtttttgtaaacgcaccgccattatatctgccgcgaaggtacgccattgcaaacgcaaggattgccccgatgccttgttcctttgccgcgagaatggcggccaacaggtcatgtttttctggcatcttcatgtcttacccccaataaggggatttgctctatttaattaggaataaggtcgattactgatagaacaaatccaggctactgtgtttagtaatcagatttgttcgtgaccgatatgcacgggcaaaacggcaggaggttgttagcgcaaaaaaaaaattccaaaaaaaaaattccaaaaaaaaaaagcgactaacaaacacaatctgatggcagcgactaacaaacacaatctgatggc

SEQ ID NO: 434 - DNA, 28 bp, artificial sequence
  polynucleotide sequence used in Example 18
gcaatatcagcaccaacagaaacaacct

SEQ ID NO: 435 - protein, 10 aa, artificial sequence
  amino acid sequence of StepII(C)
SAWSHPQFEK

SEQ ID NO: 436 - protein, 15 aa, artificial sequence
  amino acid sequence of Pro
MQRLFLLVAVMLLSG

SEQ ID NO: 437 - DNA, 22 bp, artificial sequence
  Primer
tctttaaccgccccgcctaaag

SEQ ID NO: 438 - DNA, 20 bp, artificial sequence
  Primer
cattttttgccctcgttatc

SEQ ID NO: 439 - DNA, 67 bp, artificial sequence
  Primer
aataactcaaccgatttttaagccccagcttcataaggaaaataatcgtgtaggctggagctgcttc

SEQ ID NO: 440 - DNA, 66 bp, artificial sequence
  Primer
cgcttaaacagtaaaatgccggatgataattccggcttttttatctgcatatgaatatcctcctta

SEQ ID NO: 441 - DNA, 78 bp, artificial sequence
  Hairpin
gcggggagcgtattagagttggatcggatgcagctggctactgacgtcatgacgtcagtagccagcatgcatccgatc

SEQ ID NO: 442 - protein, 239 aa, Pseudoalteromonas sp. (strain SM9913)
MGNLIPPSKQSAVTLEPTDVFSDLKSLPKPAGSIPVSVYSFRDQTGQYKPQTNVSSFSTAVTQGANSILVQALHESDWFTPVEREGLQNILTERKIIRAAQATNPNQGELPPLTTAKIILEGGIISYDTNVKTGGLGMEYFGIGASELYREDAISIYLRAVDVRTGQVLLSVATSKKVLSQEMRAGFFRYVSYKRLAEAEAGFSDNEPMSICVTQAIEKALTDLITKGIDKGLWAKQAT

SEQ ID NO: 443 - protein, 252 aa, Shewanella baltica
CSLIPKPDLNITPAEVNPLSEVMRGLQTQPGPKFPIPVAVYSFRDQTGQYKPQANVSSFSTAVTQGATSMLMQTLLDSKWFTPVEREGLQNLLTERKISNKQSGTKGDDVPVLSTARLLLEGGVISYETNTSTGGSGVEYYGIGASEMYREDQVTIYLRAVDVHTGKVMMSVSTSKRVLSQEMRAGLFRYTSLNRLAEAEIGFTTNEPVQFCVLQAIELAVAELIDKGIKQGYWSPTQVTQPVEKAQELSQS

SEQ ID NO: 444 - protein, 264 aa, Pseudomonas entomophila
CGLREPMPAEQDAETPTLTPRASTYYDLINMPRPRGRLMAVVYGFRDQTGQYKPTPASSFSTSVTQGAASMLMDALNASGWFVVLEREGLQNLLTERKIIRASQKKPDVAENIQGELPPLQAANLMLEGGIIAYDTNVRSGGEGARYLGIDISREYRVDQVTVNLRAVDVRTGQVLANVMTSKTIYSVGRSAGVFKFIEFKKLLEAEVGYTTNEPAQLCVLSAIEAAVGHLLAQGIERRLWQVAADGAGDKALLDKYLSQYQQP

SEQ ID NO: 445 - protein, 261 aa, Hafnia alvei
CAGMVATSENLEGAEATLTPRGATYQDLVSLPPPSGKIFVSVYDFRDQTGQYRPAPASTFSTAVTQGAAAMLTGSLSDSGWFIPLERVGLQNLLTERRIIRAEFERFGQPDTLPSLRAASVMLEGGIIAYESNIRTGGAGAEYFGIGASGQYQVDQVTVNLRAVEISTGEILANVTTTKTIYSKELRAGVYRFIDFSRLLEAEAGITANEPVQLAVMSAIESAVIHLIARGIENRLWNLAPGVSLQESILNDYLNAPIPML

SEQ ID NO: 446 - protein, 262 aa, Escherichia coli; identical to SEQ ID NO: 390

SEQ ID NO: 447 - protein, 263 aa, Vibrio orientalis
CSNSMTIPDADEAPTLMPRGATYQDLVQLPEPKGRILVSVYDFRDQTGQYKPQPNSNFSTAVPQGGTALLTASLLDSRWFIPLEREGLQNLLTERKIIRAAQKKGQAASNHGDDLSALSSANVVIEGGIVAYDSNIKTGGLGARYLGIGSSGKYRTDQVTVNLRAVNVRTGQILLSVTTSKTIFSHELTAGAFRFIDYKDLLEVEMGYTNNEPVNVAVMSAIDAAVIHLIVKGIGRGLWQPENKEDLQDETIQRYAKQTHQIL

SEQ ID NO: 448 - protein, 267 aa, Shewanella pealeana
CSTMSEIEQITPSSSLMPKSETYYDLIGLPAPQGSMVAAVYDFRDQTGQYKPIPSSNFSTAVPQSGTAFLAQALNDSSWFTPVEREGLQNLLTERKIVRAGLKGDAASLSQLNSAQILMEGGIVAYDTNIRTGGAGARYLGIGASGQFRVDSITVNLRAVDIRTGRLLSSVTTTKSVLSKELTAGVFKFIDAQELLESEIGYTSNEPVSLCVAQAIESAVVHMIADGIWKRAWNLADSQTGLENPILKKYWLEAHSVERVQARLEQG

SEQ ID NO: 449 - protein, 21 aa, artificial sequence
  TM1 hairpin (figure 43)
VKSGGVGARYFGIGADTQYQL

SEQ ID NO: 450 - protein, 27 aa, artificial sequence
  TM2 hairpin (figure 43)
LSYEVQAGVFRFIDYQRLLEGEVGYTS